European Patent Specification EP 4 103 719 B1, published April 1, 2026. Title: Burden-addicted production strains. Applicant: Danmarks Tekniske Universitet. The sequence listing filed with the application follows.

SEQUENCE LISTING (164 sequences)

SEQ ID NO: 1 - DNA, 2179 bp, E. coli
  gene (1)..(2179): E. coli essential gene folP-glmM
  CDS (1)..(849): folP
atgaaactctttgcccagggtacttcactggaccttagccatcctcacgtaatggggatcctcaacgtcacgcctgattccttttcggatggtggcacgcataactcgctgatagatgcggtgaaacatgcgaatctgatgatcaatgctggcgcgacgatcattgacgttggtggcgagtccacgcgcccaggggcggcggaagttagcgttgaagaagagttgcaacgtgttattcctgtggttgaggcaattgctcaacgcttcgaagtctggatctcggtcgatacatccaaaccagaagtcatccgtgagtcagcgaaagttggcgctcacattattaatgatatccgctccctttccgaacctggcgctctggaggcggctgcagaaaccggtttaccggtttgtctgatgcatatgcagggaaatccaaaaaccatgcaggaagctccgaagtatgacgatgtctttgcagaagtgaatcgctactttattgagcaaatagcacgttgcgagcaggcgggtatcgcaaaagagaaattgttgctcgaccccggattcggtttcggtaaaaatctctcccataactattcattactggcgcgcctggctgaatttcaccatttcaacctgccgctgttggtgggtatgtcacgaaaatcgatgattgggcagctgctgaacgtggggccgtccgagcgcctgagcggtagtctggcctgtgcggtcattgccgcaatgcaaggcgcgcacatcattcgtgttcatgacgtcaaagaaaccgtagaagcgatgcgggtggtggaagccactctgtctgcaaaggaaaacaaacgctatgagtaatcgtaaatatttcggtaccgatgggattcgtggtcgtgtaggggatgcgccgatcacacctgattttgtgcttaagctgggttgggccgcgggtaaagtgctggcgcgccacggctcccgtaagatcattattggtaaagacacgcgtatttctggctatatgctggagtcagcactggaagcgggtctggcggcagcgggcctttccgcactcttcactggcccgatgccaacaccggccgtggcttatctgacgcgtaccttccgcgcagaggccggaattgtgatatctgcatcgcataacccgttctacgataatggcattaaattcttctctatcgacggcaccaaactgccggatgcggtagaagaggccatcgaagcggaaatggaaaaggagatcagctgcgttgattcggcagaactgggtaaagccagccgtatcgttgatgccgcgggtcgctatatcgagttttgcaaagccacgttcccgaacgaacttagcctcagtgaactgaagattgtggtggattgtgcaaacggtgcgacttatcacatcgcgccgaacgtgctgcgcgaactgggggcgaacgttatcgctatcggttgtgagccaaacggtgtaaacatcaatgccgaagtgggggctaccgacgttcgcgcgctccaggctcgtgtgctggctgaaaaagcggatctcggtattgccttcgacggcgatggcgatcgcgtgattatggttgaccatgaaggcaataaagtcgatggcgatcagatcatgtatatcatcgcgcgtgaaggtcttcgtcagggccagctgcgtggtggcgctgtgggtacattgatgagcaacatggggcttgaactggcgctgaaacagttaggaattccatttgcgcgcgcgaaagtgggtgaccgctacgtactggaaaaaatgcaggagaaaggctggcgtatcggtgcagagaattccggtcatgtgatcctgctggataaaactactaccggtgacggcatcgttgctggcttgcaggtgctggcggctatggcacgtaaccatatgagcctgcacgacctttgcagcggcatgaaaatgttcccgcagattctggttaacgtacgttacaccgcaggtagcggcgatccacttgagcatgagtcagttaaagccgtgaccgcagaggttgaagctgcgctgggcaaccgtggacgcgtgttgctgcgtaaatccggcaccgaaccgttaattcgcgtgatggtggaaggcgaagacgaagcgcaggtgactgaatttgcacaccgcatcgccgatgcagtaaaagccgtttaa

SEQ ID NO: 2 - protein, 282 aa, E. coli
MKLFAQGTSLDLSHPHVMGILNVTPDSFSDGGTHNSLIDAVKHANLMINAGATIIDVGGESTRPGAAEVSVEEELQRVIPVVEAIAQRFEVWISVDTSKPEVIRESAKVGAHIINDIRSLSEPGALEAAAETGLPVCLMHMQGNPKTMQEAPKYDDVFAEVNRYFIEQIARCEQAGIAKEKLLLDPGFGFGKNLSHNYSLLARLAEFHHFNLPLLVGMSRKSMIGQLLNVGPSERLSGSLACAVIAAMQGAHIIRVHDVKETVEAMRVVEATLSAKENKRYE

SEQ ID NO: 3 - DNA, 1338 bp, E. coli
  CDS (1)..(1338): E. coli essential gene glmM
atgagtaatcgtaaatatttcggtaccgatgggattcgtggtcgtgtaggggatgcgccgatcacacctgattttgtgcttaagctgggttgggccgcgggtaaagtgctggcgcgccacggctcccgtaagattattattggtaaagacacgcgtatttctggctatatgctggagtcagcactggaagcgggtctggcggcagcgggcctttccgcactcttcactggcccgatgccaacaccggccgtggcttatctgacgcgtaccttccgcgcagaggccggaattgtgatatctgcatcgcataacccgttctacgataatggcattaaattcttctctatcgacggcaccaaactgccggatgcggtagaagaggccatcgaagcggaaatggaaaaggagatcagctgcgttgattcggcagaactgggtaaagccagccgtatcgttgatgccgcgggtcgctatatcgagttttgcaaagccacgttcccgaacgaacttagcctcagtgaactgaagattgtggtggattgtgcaaacggtgcgacttatcacatcgcgccgaacgtgctgcgcgaactgggggcgaacgttatcgctatcggttgtgagccaaacggtgtaaacatcaatgccgaagtgggggctaccgacgttcgcgcgctccaggctcgtgtgctggctgaaaaagcggatctcggtattgccttcgacggcgatggcgatcgcgtgattatggttgaccatgaaggcaataaagtcgatggcgatcagatcatgtatatcatcgcgcgtgaaggtcttcgtcagggccagctgcgtggtggcgctgtgggtacattgatgagcaacatggggcttgaactggcgctgaaacagttaggaattccatttgcgcgcgcgaaagtgggtgaccgctacgtactggaaaaaatgcaggagaaaggctggcgtatcggtgcagagaattccggtcatgtgatcctgctggataaaactactaccggtgacggcatcgttgctggcttgcaggtgctggcggcgatggcacgtaaccatatgagcctgcacgacctttgcagcggcatgaaaatgttcccgcagattctggttaacgtacgttacaccgcaggtagcggcgatccacttgagcatgagtcagttaaagccgtgaccgcagaggttgaagctgcgctgggcaaccgtggacgcgtgttgctgcgtaaatccggcaccgaaccgttaattcgcgtgatggtggaaggcgaagacgaagcgcaggtgactgaatttgcacaccgcatcgccgatgcagtaaaagccgtttaa

SEQ ID NO: 4 - protein, 445 aa, E. coli
MSNRKYFGTDGIRGRVGDAPITPDFVLKLGWAAGKVLARHGSRKIIIGKDTRISGYMLESALEAGLAAAGLSALFTGPMPTPAVAYLTRTFRAEAGIVISASHNPFYDNGIKFFSIDGTKLPDAVEEAIEAEMEKEISCVDSAELGKASRIVDAAGRYIEFCKATFPNELSLSELKIVVDCANGATYHIAPNVLRELGANVIAIGCEPNGVNINAEVGATDVRALQARVLAEKADLGIAFDGDGDRVIMVDHEGNKVDGDQIMYIIAREGLRQGQLRGGAVGTLMSNMGLELALKQLGIPFARAKVGDRYVLEKMQEKGWRIGAENSGHVILLDKTTTGDGIVAGLQVLAAMARNHMSLHDLCSGMKMFPQILVNVRYTAGSGDPLEHESVKAVTAEVEAALGNRGRVLLRKSGTEPLIRVMVEGEDEAQVTEFAHRIADAVKAV

SEQ ID NO: 5 - DNA, 858 bp, E. coli
  CDS (1)..(858): E. coli essential gene murI
atggctaccaaactgcaggacgggaatacaccttgtctggcagctacaccttctgaaccacgtcccaccgtgctggtgtttgactccggcgtcggtgggttgtcggtctatgacgagatccggcatctcttaccggatctccattacatttatgctttcgataacgtcgctttcccgtatggcgaaaaaagcgaagcgtttattgttgagcgagtggtggcaattgtcaccgcggtgcaagaacgttatccccttgcgctggctgtggtcgcttgcaacactgccagtaccgtttcacttcctgcattacgcgaaaagttcgacttcccggttgttggtgtcgtgccggcgattaaacctgctgcacgtctgacggcaaatggcattgtcggattactggcaacccgcggaacagttaaacgttcttatactcatgagctgatcgcgcgtttcgctaatgaatgccagatagaaatgctgggctcggcagagatggttgagttggctgaagcgaagctacatggcgaagatgtttctctggatgcactaaaacgtatcctacgcccgtggttaagaatgaaagagccgccagataccgttgtattgggttgcacccatttccctctactacaagaagaactgttacaagtgctgccagagggaacccggctggtggattctggcgcagcgattgctcgccgaacggcctggttgttagaacatgaagccccggatgcaaaatctgccgatgcgaatattgccttttgtatggcaatgacgccaggagctgaacaattattgcccgttttacagcgttacggcttcgaaacgctcgaaaaactggcagttttaggctga

SEQ ID NO: 6 - protein, 285 aa, E. coli
MATKLQDGNTPCLAATPSEPRPTVLVFDSGVGGLSVYDEIRHLLPDLHYIYAFDNVAFPYGEKSEAFIVERVVAIVTAVQERYPLALAVVACNTASTVSLPALREKFDFPVVGVVPAIKPAARLTANGIVGLLATRGTVKRSYTHELIARFANECQIEMLGSAEMVELAEAKLHGEDVSLDALKRILRPWLRMKEPPDTVVLGCTHFPLLQEELLQVLPEGTRLVDSGAAIARRTAWLLEHEAPDAKSADANIAFCMAMTPGAEQLLPVLQRYGFETLEKLAVLG

SEQ ID NO: 7 - DNA, 1104 bp, E. coli
  CDS (1)..(1104): E. coli essential gene asd
atgaaaaatgttggttttatcggctggcgcggtatggtcggctccgttctcatgcaacgcatggttgaagagcgcgacttcgacgccattcgccctgtctacttttctacttctcagcttggtcaggctgcgccgtcttttggcggaaccactggcacacttcaggatgcctttgatctggaggcgctaaaggccctcgatatcattgtgacctgtcagggcggcgattataccaacgaaatctatccaaagcttcgtgaaagcggatggcagggttactggattgacgcagcatcgtctctgcgcatgaaagatgacgccatcatcattcttgaccccgtcaatcaggacgtcattaccgacggattaaataatggcatcaggacttttgttggcggtaactgtaccgtaagcctgatgttgatgtcgttgggtggtttattcgccaatgatcttgttgattgggtgtccgttgcaacctaccaggccgcttccggcggtggtgcgcgacatatgcgtgagttattaacccagatgggccatctgtatggccatgtagcagatgaactcgcgaccccgtcctctgctattctcgatatcgaacgcaaagtcacaaccttaacccgtagcggtgagctgccggtggataactttggcgtgccgctggcgggtagcctgattccgtggatcgacaaacagctcgataacggtcagagccgcgaagagtggaaagggcaggcggaaaccaacaagatcctcaacacatcttccgtaattccggtagatggtttatgtgtgcgtgtcggggcattgcgctgccacagccaggcattcactattaaattgaaaaaagatgtgtcgattccgaccgtggaagaactgctggctgcgcacaatccgtgggcgaaagtcgttccgaacgatcgggaaatcactatgcgtgagctaaccccagctgccgttaccggcacgctgaccacgccggtaggccgcctgcgtaagctgaatatgggaccagagttcctgtcagcctttaccgtgggcgaccagctgctgtggggggccgcggagccgctgcgtcggatgcttcgtcaactggcgtaa

SEQ ID NO: 8 - protein, 367 aa, E. coli
MKNVGFIGWRGMVGSVLMQRMVEERDFDAIRPVYFSTSQLGQAAPSFGGTTGTLQDAFDLEALKALDIIVTCQGGDYTNEIYPKLRESGWQGYWIDAASSLRMKDDAIIILDPVNQDVITDGLNNGIRTFVGGNCTVSLMLMSLGGLFANDLVDWVSVATYQAASGGGARHMRELLTQMGHLYGHVADELATPSSAILDIERKVTTLTRSGELPVDNFGVPLAGSLIPWIDKQLDNGQSREEWKGQAETNKILNTSSVIPVDGLCVRVGALRCHSQAFTIKLKKDVSIPTVEELLAAHNPWAKVVPNDREITMRELTPAAVTGTLTTPVGRLRKLNMGPEFLSAFTVGDQLLWGAAEPLRRMLRQLA

SEQ ID NO: 9 - DNA, 1104 bp, E. coli; identical to SEQ ID NO: 7
  CDS (1)..(1104): E. coli essential gene thyA

SEQ ID NO: 10 - protein, 367 aa, E. coli; identical to SEQ ID NO: 8

SEQ ID NO: 11 - DNA, 1842 bp, E. coli
  CDS (1)..(1842): E. coli essential gene rpoD
atggagcaaaacccgcagtcacagctgaaacttcttgtcacccgtggtaaggagcaaggctatctgacctatgccgaggtcaatgaccatctgccggaagatatcgtcgattcagatcagatcgaagacatcatccaaatgatcaacgacatgggcattcaggtgatggaagaagcaccggatgccgatgatctgatgctggctgaaaacaccgcggacgaagatgctgccgaagccgccgcgcaggtgctttccagcgtggaatctgaaatcgggcgcacgactgacccggtacgcatgtacatgcgtgaaatgggcaccgttgaactgttgacccgcgaaggcgaaattgacatcgctaagcgtattgaagacgggatcaaccaggttcaatgctccgttgctgaatatccggaagcgatcacctatctgctggaacagtacgatcgtgttgaagcagaagaagcgcgtctgtccgatctgatcaccggctttgttgacccgaacgcagaagaagatctggcacctaccgccactcacgtcggttctgagctttcccaggaagatctggacgatgacgaagatgaagacgaagaagatggcgatgacgacagcgccgatgatgacaacagcatcgacccggaactggctcgcgaaaaatttgcggaactacgcgctcagtacgttgtaacgcgtgacaccatcaaagcgaaaggtcgcagtcacgctaccgctcaggaagagatcctgaaactgtctgaagtattcaaacagttccgcctggtgccgaagcagtttgactacctggtcaacagcatgcgcgtcatgatggaccgcgttcgtacgcaagaacgtctgatcatgaagctctgcgttgagcagtgcaaaatgccgaagaaaaacttcattaccctgtttaccggcaacgaaaccagcgatacctggttcaacgcggcaattgcgatgaacaagccgtggtcggaaaaactgcacgatgtctctgaagaagtgcatcgcgccctgcaaaaactgcagcagattgaagaagaaaccggcctgaccatcgagcaggttaaagatatcaaccgtcgtatgtccatcggtgaagcgaaagcccgccgtgcgaagaaagagatggttgaagcgaacttacgtctggttatttctatcgctaagaaatacaccaaccgtggcttgcagttccttgacctgattcaggaaggcaacatcggtctgatgaaagcggttgataaattcgaataccgccgtggttacaagttctccacctacgcaacctggtggatccgtcaggcgatcacccgctctatcgcggatcaggcgcgcaccatccgtattccggtgcatatgattgagaccatcaacaagctcaaccgtatttctcgccagatgctgcaagagatgggccgtgaaccgacgccggaagaactggctgaacgtatgctgatgccggaagacaagatccgcaaagtgctgaagatcgccaaagagccaatctccatggaaacgccgatcggtgatgatgaagattcgcatctgggggatttcatcgaggataccaccctcgagctgccgctggattctgcgaccaccgaaagcctgcgtgcggcaacgcacgacgtgctggctggcctgaccgcgcgtgaagcaaaagttctgcgtatgcgtttcggtatcgatatgaacaccgaccacacgctggaagaagtgggtaaacagttcgacgttacccgcgaacgtatccgtcagatcgaagcgaaggcgctgcgcaaactgcgtcacccgagccgttctgaagtgctgcgtagcttcctggacgattaa

SEQ ID NO: 12 - protein, 613 aa, E. coli
MEQNPQSQLKLLVTRGKEQGYLTYAEVNDHLPEDIVDSDQIEDIIQMINDMGIQVMEEAPDADDLMLAENTADEDAAEAAAQVLSSVESEIGRTTDPVRMYMREMGTVELLTREGEIDIAKRIEDGINQVQCSVAEYPEAITYLLEQYDRVEAEEARLSDLITGFVDPNAEEDLAPTATHVGSELSQEDLDDDEDEDEEDGDDDSADDDNSIDPELAREKFAELRAQYVVTRDTIKAKGRSHATAQEEILKLSEVFKQFRLVPKQFDYLVNSMRVMMDRVRTQERLIMKLCVEQCKMPKKNFITLFTGNETSDTWFNAAIAMNKPWSEKLHDVSEEVHRALQKLQQIEEETGLTIEQVKDINRRMSIGEAKARRAKKEMVEANLRLVISIAKKYTNRGLQFLDLIQEGNIGLMKAVDKFEYRRGYKFSTYATWWIRQAITRSIADQARTIRIPVHMIETINKLNRISRQMLQEMGREPTPEELAERMLMPEDKIRKVLKIAKEPISMETPIGDDEDSHLGDFIEDTTLELPLDSATTESLRAATHDVLAGLTAREAKVLRMRFGIDMNTDHTLEEVGKQFDVTRERIRQIEAKALRKLRHPSRSEVLRSFLDD

SEQ ID NO: 13 - DNA, 546 bp, E. coli
  CDS (1)..(546): E. coli essential gene nusG
atgtctgaagctcctaaaaagcgctggtacgtcgttcaggcgttttccggttttgaaggccgcgtagcaacgtcgctgcgtgagcatatcaaattacacaacatggaagatttgtttggtgaagtcatggtaccaaccgaagaagtggttgaaatccgtggcggtcagcgtcgcaaaagcgaacgtaaattcttccctggctacgtcctcgttcagatggtgatgaacgacgcgagctggcacctggtgcgcagcgtaccgcgtgtgatgggcttcatcggcggtacttccgatcgtcctgcgccaatcagcgataaagaagtcgatgcgattatgaaccgcctgcagcaggttggtgataagccgcgtccgaaaacgctgtttgaaccgggtgaaatggtccgtgttaatgatggtccgttcgctgacttcaacggtgttgttgaagaagtggattacgagaaatctcgtctgaaagtgtctgtttctatcttcggtcgtgcgaccccggtagagctggacttcagccaggttgaaaaagcctaa

SEQ ID NO: 14 - protein, 181 aa, E. coli
MSEAPKKRWYVVQAFSGFEGRVATSLREHIKLHNMEDLFGEVMVPTEEVVEIRGGQRRKSERKFFPGYVLVQMVMNDASWHLVRSVPRVMGFIGGTSDRPAPISDKEVDAIMNRLQQVGDKPRPKTLFEPGEMVRVNDGPFADFNGVVEEVDYEKSRLKVSVSIFGRATPVELDFSQVEKA

SEQ ID NO: 15 - DNA, 216 bp, E. coli
  CDS (1)..(216): E. coli essential gene rpsU
atgccggtaattaaagtacgtgaaaacgagccgttcgacgtagctctgcgtcgcttcaagcgttcctgcgaaaaagcaggtgttctggcggaagttcgtcgtcgtgagttctatgaaaaaccgactaccgaacgtaagcgcgctaaagcttctgcagtgaaacgtcacgcgaagaaactggctcgcgaaaacgcacgccgcactcgtctgtactaa

SEQ ID NO: 16 - protein, 71 aa, E. coli
MPVIKVRENEPFDVALRRFKRSCEKAGVLAEVRRREFYEKPTTERKRAKASAVKRHAKKLARENARRTRLY

SEQ ID NO: 17 - DNA, 216 bp, E. coli; identical to SEQ ID NO: 15
  CDS (1)..(216): E. coli essential gene accD

SEQ ID NO: 18 - protein, 71 aa, E. coli; identical to SEQ ID NO: 16

SEQ ID NO: 19 - DNA, 216 bp, E. coli; identical to SEQ ID NO: 15
  CDS (1)..(216): E coli essential gene degS

SEQ ID NO: 20 - protein, 71 aa, E. coli; identical to SEQ ID NO: 16

SEQ ID NO: 21 - DNA, 531 bp, E. coli
  CDS (1)..(531): E. coli essential gene fldA
atggctatcactggcatctttttcggcagcgacaccggtaataccgaaaatatcgcaaaaatgattcaaaaacagcttggtaaagacgttgccgatgtccatgacattgcaaaaagcagcaaagaagatctggaagcttatgacattctgctgctgggcatcccaacctggtattacggcgaagcgcagtgtgactgggatgacttcttcccgactctcgaagagattgatttcaatggcaaactggttgcgctgtttggttgtggtgaccaggaagattacgccgaatatttctgcgacgcattgggcaccatccgcgacatcattgaaccgcgcggtgcaaccatcgttggtcactggccaactgcgggctatcatttcgaagcatcaaaaggtctggcagatgacgaccactttgtcggtctggctatcgacgaagaccgtcagccggaactgaccgctgaacgtgtagaaaaatgggttaaacagatttctgaagagttgcatctcgacgaaattctcaatgcctga

SEQ ID NO: 22 - protein, 176 aa, E. coli
MAITGIFFGSDTGNTENIAKMIQKQLGKDVADVHDIAKSSKEDLEAYDILLLGIPTWYYGEAQCDWDDFFPTLEEIDFNGKLVALFGCGDQEDYAEYFCDALGTIRDIIEPRGATIVGHWPTAGYHFEASKGLADDDHFVGLAIDEDRQPELTAERVEKWVKQISEELHLDEILNA

SEQ ID NO: 23 - DNA, 960 bp, E. coli
  CDS (1)..(960): E. coli essential gene ftsN
gtggcacaacgagattatgtacgccgcagccaaccggcaccttcgcggcgaaaaaagagcacctcacggaaaaagcaacgaaatctgcctgcggtttctcccgctatggtcgctattgctgccgccgttcttgtgacctttatcggtggtctgtacttcattacgcatcacaagaaagaagagtccgagacgctgcaaagccagaaagtgaccggaaacggactaccaccaaaaccagaagaacgctggcgctacattaaagagctggaaagtcgccagccgggagtgcgtgcgcccacagaaccttctgccggtggtgaagtgaaaacgccggagcaactgacaccagaacaacgtcagcttcttgaacaaatgcaggctgatatgcgccagcagccaacgcagctggttgaagttccgtggaatgaacagacgccggaacagcgtcagcaaacgctacagcgccaacgtcaggcgcagcaattagcggaacagcaacgcctggctcagcagtcgcgtacgactgaacaaagctggcagcagcagacgcgtacgtcgcaagccgcaccggtacaggcgcaaccgcgccagtctaaaccggcttcttctcagcagccgtaccaggatctgctgcaaactcctgcgcacacgactgcgcagtcgaagccgcagcaagctgcgccagttgctcgtgccgctgacgcgccaaaaccgacggcggagaaaaaagacgaacgccgctggatggtgcagtgcggttcgttcagaggcgcggaacaggcagagacggtacgtgctcagctggcgttcgaaggctttgactcgaaaatcaccaccaacaatggctggaatcgtgtggtcattggcccggtgaaaggcaaagagaacgcagacagcaccctcaatcggttgaagatggcgggccatacaaactgcattcggctcgccgccgggggttga

SEQ ID NO: 24 - protein, 319 aa, E. coli
VAQRDYVRRSQPAPSRRKKSTSRKKQRNLPAVSPAMVAIAAAVLVTFIGGLYFITHHKKEESETLQSQKVTGNGLPPKPEERWRYIKELESRQPGVRAPTEPSAGGEVKTPEQLTPEQRQLLEQMQADMRQQPTQLVEVPWNEQTPEQRQQTLQRQRQAQQLAEQQRLAQQSRTTEQSWQQQTRTSQAAPVQAQPRQSKPASSQQPYQDLLQTPAHTTAQSKPQQAAPVARAADAPKPTAEKKDERRWMVQCGSFRGAEQAETVRAQLAFEGFDSKITTNNGWNRVVIGPVKGKENADSTLNRLKMAGHTNCIRLAAGG

SEQ ID NO: 25 - DNA, 1935 bp, E. coli
  CDS (1)..(1935): E. coli essential gene hflB
atggcgaaaaacctaatactctggctggtcattgccgttgtgctgatgtcagtattccagagctttgggcccagcgagtctaatggccgtaaggtggattactctaccttcctacaagaggtcaataacgaccaggttcgtgaagcgcgtatcaacggacgtgaaatcaacgttaccaagaaagatagtaaccgttataccacttacattccggttcaggatccgaaattactggataacctgttgaccaagaacgtcaaggttgtcggtgaaccgcctgaagaaccaagcctgctggcttctatcttcatctcctggttcccgatgctgttgctgattggtgtctggatcttcttcatgcgtcaaatgcagggcggcggtggcaaaggtgccatgtcgtttggtaagagcaaagcgcgcatgctgacggaagatcagatcaaaacgacctttgctgacgttgcgggctgcgacgaagcaaaagaagaagttgctgaactggttgagtatctgcgcgagccgagccgcttccagaaactcggcggtaagatcccgaaaggcgtcttgatggtcggtcctccgggtaccggtaaaacgctgctggcgaaagcgattgcaggcgaagcgaaagttccgttctttactatctccggttctgacttcgtagaaatgttcgtcggtgtgggtgcatcccgtgttcgtgacatgttcgaacaggcgaagaaagcggcaccgtgcatcatctttatcgatgaaatcgacgccgtaggccgccagcgtggcgctggtctgggcggtggtcacgatgaacgtgaacagactctgaaccagatgctggttgagatggatggcttcgaaggtaacgaaggtatcatcgttatcgccgcgactaaccgtccggacgttctcgacccggccctgctgcgtcctggccgtttcgaccgtcaggttgtggtcggcttgccagatgttcgcggtcgtgagcagatcctgaaagttcacatgcgtcgcgtaccattggcacccgatatcgacgcggcaatcattgcccgtggtactcctggtttctccggtgctgacctggcgaacctggtgaacgaagcggcactgttcgctgctcgtggcaacaaacgcgttgtgtcgatggttgagttcgagaaagcgaaagacaaaatcatgatgggtgcggaacgtcgctccatggtgatgacggaagcgcagaaagaatcgacggcttaccacgaagcgggtcatgcgattatcggtcgcctggtgccggaacacgatccggtgcacaaagtgacgattatcccacgcggtcgtgcgctgggtgtgactttcttcttgcctgagggcgacgcaatcagcgccagccgtcagaaactggaaagccagatttctacgctgtacggtggtcgtctggcagaagagatcatctacgggccggaacatgtatctaccggtgcgtccaacgatattaaagttgcgaccaacctggcacgtaacatggtgactcagtggggcttctctgagaaattgggtccactgctgtacgcggaagaagaaggtgaagtgttcctcggccgtagcgtagcgaaagcgaaacatatgtccgatgaaactgcacgtatcatcgaccaggaagtgaaagcactgattgagcgtaactataatcgtgcgcgtcagcttctgaccgacaatatggatattctgcatgcgatgaaagatgctctcatgaaatatgagactatcgacgcaccgcagattgatgacctgatggcacgtcgcgatgtacgtccgccagcgggctgggaagaaccaggcgcttctaacaattctggcgacaatggtagtccaaaggctcctcgtccggttgatgaaccgcgtacgccgaacccgggtaacaccatgtcagagcagttaggcgacaagtaa

SEQ ID NO: 26 - protein, 644 aa, E. coli
MAKNLILWLVIAVVLMSVFQSFGPSESNGRKVDYSTFLQEVNNDQVREARINGREINVTKKDSNRYTTYIPVQDPKLLDNLLTKNVKVVGEPPEEPSLLASIFISWFPMLLLIGVWIFFMRQMQGGGGKGAMSFGKSKARMLTEDQIKTTFADVAGCDEAKEEVAELVEYLREPSRFQKLGGKIPKGVLMVGPPGTGKTLLAKAIAGEAKVPFFTISGSDFVEMFVGVGASRVRDMFEQAKKAAPCIIFIDEIDAVGRQRGAGLGGGHDEREQTLNQMLVEMDGFEGNEGIIVIAATNRPDVLDPALLRPGRFDRQVVVGLPDVRGREQILKVHMRRVPLAPDIDAAIIARGTPGFSGADLANLVNEAALFAARGNKRVVSMVEFEKAKDKIMMGAERRSMVMTEAQKESTAYHEAGHAIIGRLVPEHDPVHKVTIIPRGRALGVTFFLPEGDAISASRQKLESQISTLYGGRLAEEIIYGPEHVSTGASNDIKVATNLARNMVTQWGFSEKLGPLLYAEEEGEVFLGRSVAKAKHMSDETARIIDQEVKALIERNYNRARQLLTDNMDILHAMKDALMKYETIDAPQIDDLMARRDVRPPAGWEEPGASNNSGDNGSPKAPRPVDEPRTPNPGNTMSEQLGDK

SEQ ID NO: 27 - DNA, 612 bp, E. coli
  CDS (1)..(612): E. coli essential gene lolA
atgaaaaaaattgccatcacctgtgcattactctcaagcttagtagcaagcagcgtttgggctgatgccgcaagcgatctgaaaagccgcctggataaagtcagcagcttccacgccagcttcacacaaaaagtgactgacggtagcggcgcggcggtgcaggaaggtcagggcgatctgtgggtgaaacgtccaaacttattcaactggcatatgacacaacctgatgaaagcattctggtttctgacggtaaaacactgtggttctataacccgttcgttgagcaagctacggcaacctggctgaaagatgccaccggtaatacgccgtttatgctgattgcccgcaaccagtccagcgactggcagcagtacaatatcaaacagaatggcgatgactttgtcctgacgccgaaagccagcaatggcaatctgaagcagttcaccattaacgtgggacgtgatggcacaatccatcagtttagcgcggtggagcaggacgatcagcgcagcagttatcaactgaaatcccagcaaaatggggctgtggatgcagcgaaatttaccttcaccccgccgcaaggcgtcacggtagatgatcaacgtaagtag

SEQ ID NO: 28 - protein, 203 aa, E. coli
MKKIAITCALLSSLVASSVWADAASDLKSRLDKVSSFHASFTQKVTDGSGAAVQEGQGDLWVKRPNLFNWHMTQPDESILVSDGKTLWFYNPFVEQATATWLKDATGNTPFMLIARNQSSDWQQYNIKQNGDDFVLTPKASNGNLKQFTINVGRDGTIHQFSAVEQDDQRSSYQLKSQQNGAVDAAKFTFTPPQGVTVDDQRK

SEQ ID NO: 29 - DNA, 1083 bp, E. coli
  CDS (1)..(1083): E. coli essential gene mraY
atgttagtttggctggccgaacatttggtcaaatattattccggctttaacgtcttttcctatctgacgtttcgcgccatcgtcagcctgctgaccgcgctgttcatctcattgtggatgggcccgcgtatgattgctcatttgcaaaaactttcctttggtcaggtggtgcgtaacgacggtcctgaatcacacttcagcaagcgcggtacgccgaccatgggcgggattatgatcctgacggcgattgtgatctccgtactgctgtgggcttacccgtccaatccgtacgtctggtgcgtgttggtggtgctggtaggttacggtgttattggctttgttgatgattatcgcaaagtggtgcgtaaagacaccaaagggttgatcgctcgttggaagtatttctggatgtcggtcattgcgctgggtgtcgccttcgccctgtaccttgccggcaaagacacgcccgcaacgcagctggtggtcccattctttaaagatgtgatgccgcagctggggctgttctacattctgctggcttacttcgtcattgtgggtactggcaacgcggtaaacctgaccgatggtctcgacggcctggcaattatgccgaccgtatttgtcgccggtggttttgcgctggtggcgtgggcgaccggcaatatgaactttgccagctacttgcatataccgtatctgcgacacgccggggaactggttattgtctgtaccgcgatagtcggggcaggactgggcttcctgtggtttaacacctatccggcgcaggtctttatgggcgatgtaggttcgctggcgttaggtggtgcgttaggcattatcgccgtactgctacgtcaggaattcctgctggtgattatggggggcgtgttcgtggtagaaacgctttctgtcatcctgcaggtcggctcctttaaactgcgcggacaacgtattttccgcatggcaccgattcatcaccactatgaactgaaaggctggccggaaccgcgcgtcattgtgcgtttctggattatttcgctgatgctggttctgattggtctggcaacgctgaaggtacgttaa

SEQ ID NO: 30 - protein, 360 aa, E. coli
MLVWLAEHLVKYYSGFNVFSYLTFRAIVSLLTALFISLWMGPRMIAHLQKLSFGQVVRNDGPESHFSKRGTPTMGGIMILTAIVISVLLWAYPSNPYVWCVLVVLVGYGVIGFVDDYRKVVRKDTKGLIARWKYFWMSVIALGVAFALYLAGKDTPATQLVVPFFKDVMPQLGLFYILLAYFVIVGTGNAVNLTDGLDGLAIMPTVFVAGGFALVAWATGNMNFASYLHIPYLRHAGELVIVCTAIVGAGLGFLWFNTYPAQVFMGDVGSLALGGALGIIAVLLRQEFLLVIMGGVFVVETLSVILQVGSFKLRGQRIFRMAPIHHHYELKGWPEPRVIVRFWIISLMLVLIGLATLKVR

SEQ ID NO: 31 - DNA, 489 bp, E. coli
  CDS (1)..(489): E. coli essential gene mreD
gtggcgagctatcgtagccagggacgctgggtaatctggctctctttcctcattgcgctgttgctgcaaatcatgccctggccggataacctgattgttttccggccaaactgggtgttactcatcttgttgtattggatcctggccttgcctcatcgcgtaaatgtgggcacaggttttgtgatgggtgccatactggatctgatcagcggctcgacgcttggcgtacgcgtattggcgatgagcatcattgcttacctggtggcgctgaaataccagcttttccgcaacctcgcattatggcagcaggcgctggtcgtcatgttgctttcgctggtggtggatattattgttttctgggcagagtttttagtgattaacgtctctttcagaccggaagtgttctggagtagtgtagtcaatggggtgctctggccgtggattttcttgctgatgcgcaaagtccgtcagcagtttgcagtgcaataa

SEQ ID NO: 32 - protein, 162 aa, E. coli
VASYRSQGRWVIWLSFLIALLLQIMPWPDNLIVFRPNWVLLILLYWILALPHRVNVGTGFVMGAILDLISGSTLGVRVLAMSIIAYLVALKYQLFRNLALWQQALVVMLLSLVVDIIVFWAEFLVINVSFRPEVFWSSVVNGVLWPWIFLLMRKVRQQFAVQ

SEQ ID NO: 33 - DNA, 1260 bp, E. coli
  CDS (1)..(1260): E. coli essential gene murA
atggataaatttcgtgttcaggggccaacgaagctccagggcgaagtcacaatttccggcgctaaaaatgctgctctgcctatcctttttgccgctctactggcggaagaaccggtagagatccagaacgtcccgaaactgaaagacgtcgatacatcaatgaagctgctaagccagctgggtgcgaaagtagaacgtaatggttctgtgcatattgatgcccgcgacgttaatgtattctgcgcaccttacgatctggttaaaaccatgcgtgcttctatctgggcactggggccgctggtagcgcgctttggtcaggggcaagtttcactacctggcggttgtacgatcggtgcgcgtccggttgatctacacatttctggcctcgaacaattaggcgcgaccatcaaactggaagaaggttacgttaaagcttccgtcgatggtcgtctgaaaggcgcacatatcgtgatggataaagtcagcgttggcgcaacggtgaccatcatgtgtgctgcaaccctggcggaaggcaccacgattattgaaaacgcagcgcgtgaaccggaaatcgtcgataccgcgaacttcctgattacgctgggtgcgaaaattagcggtcagggcaccgatcgtatcgtcatcgaaggtgtggaacgtttaggcggcggtgtctatcgcgtgctgccggatcgtatcgaaaccggtacattcctggtggcggcggcgatttctcgcggcaaaattatctgccgtaacgcgcagccagatactctcgacgccgtgctggcgaaactgcgtgacgctggagcggacatcgaagtcggcgaagactggattagcctggatatgcatggcaaacgtccgaaggctgttaacgtacgtaccgcgccgcatccggcattcccgaccgatatgcaggcccagttcacgctgttgaacctggtggcagaagggactggattcatcaccgaaacggtctttgaaaaccgctttatgcatgtgccagagctgagccgtatgggcgcgcacgccgaaatcgaaagcaataccgttatttgtcacggtgttgaaaaactttctggcgcacaggttatggcaaccgatctgcgtgcatcagcaagcctggtgctggctggctgtattgcggaagggacgacggtggttgatcgtatttatcacatcgatcgtggctacgaacgcattgaagacaaactgcgcgctttaggtgcaaatattgagcgtgtgaaaggcgagtaa

SEQ ID NO: 34 - protein, 419 aa, E. coli
MDKFRVQGPTKLQGEVTISGAKNAALPILFAALLAEEPVEIQNVPKLKDVDTSMKLLSQLGAKVERNGSVHIDARDVNVFCAPYDLVKTMRASIWALGPLVARFGQGQVSLPGGCTIGARPVDLHISGLEQLGATIKLEEGYVKASVDGRLKGAHIVMDKVSVGATVTIMCAATLAEGTTIIENAAREPEIVDTANFLITLGAKISGQGTDRIVIEGVERLGGGVYRVLPDRIETGTFLVAAAISRGKIICRNAQPDTLDAVLAKLRDAGADIEVGEDWISLDMHGKRPKAVNVRTAPHPAFPTDMQAQFTLLNLVAEGTGFITETVFENRFMHVPELSRMGAHAEIESNTVICHGVEKLSGAQVMATDLRASASLVLAGCIAEGTTVVDRIYHIDRGYERIEDKLRALGANIERVKGE

SEQ ID NO: 35 - DNA, 1029 bp, E. coli
  CDS (1)..(1029): E. coli essential gene murB
atgaaccactccttaaaaccctggaacacatttggcattgatcataatgctcagcacattgtatgtgccgaagacgaacaacaattactcaatgcctggcagcatgcaaccgcagaaggacaacccgttcttattctgggtgaaggaagtaatgtactttttctggaagactatcgcggcacggtgatcatcaaccggatcaaaggtatcgaaattcatgatgaacctgatgcgtggtatttacatgtaggagccggagaaaactggcatcgcctggtaaaatacactttgcaggaaggtatgcctggtctggaaaatctggcattaattcctggttgtgtcggctcatcacctatccagaatattggtgcttatggcgtagaattacagcgagtttgcgcttatgttgattgtgttgaactggcgacaggcaagcaagtgcgcttaactgccaaagagtgccgttttggctatcgcgacagtatttttaaacatgaataccaggatcgcttcgccattgtagccgtaggtctgcgtctgccaaaagagtggcaacctgtactaacgtatggtgacttaactcgtctggatcctacaacagtaacgccacagcaagtatttaatgcggtgtgtcatatgcgcaccaccaaactccctgatccaaaagtgaatggcaatgccggtagtttcttcaaaaaccctgttgtatctgccgaaacggctgaagcattactgtcacaatttccaacagcaccaaattacccccaggcggatggttcagtaaaactggcagcaggttggcttattgatcagtgccagctaaaagggatgcaaatgggtggggctgcggtgcaccgtcaacaggcgttagttctcattaatgaagacaatgcaaaaagcgaagatgtggtgcaactggcacaccatgtaagacaaaaagtgggtgaaaaatttaatgtctggcttgagcctgaagtccgctttattggtgcatcaggtgaagtgagcgcagtggagacaatttcatga

SEQ ID NO: 36 - protein, 342 aa, E. coli
MNHSLKPWNTFGIDHNAQHIVCAEDEQQLLNAWQHATAEGQPVLILGEGSNVLFLEDYRGTVIINRIKGIEIHDEPDAWYLHVGAGENWHRLVKYTLQEGMPGLENLALIPGCVGSSPIQNIGAYGVELQRVCAYVDCVELATGKQVRLTAKECRFGYRDSIFKHEYQDRFAIVAVGLRLPKEWQPVLTYGDLTRLDPTTVTPQQVFNAVCHMRTTKLPDPKVNGNAGSFFKNPVVSAETAEALLSQFPTAPNYPQADGSVKLAAGWLIDQCQLKGMQMGGAAVHRQQALVLINEDNAKSEDVVQLAHHVRQKVGEKFNVWLEPEVRFIGASGEVSAVETIS

SEQ ID NO: 37 - DNA, 1359 bp, E. coli
  CDS (1)..(1359): E. coli essential gene murF
atgattagcgtaacccttagccaacttaccgacattctcaacggtgaactgcaaggtgcagatatcacccttgatgctgtaaccactgatacccgaaaactgacgccgggctgcctgtttgttgccctgaaaggcgaacgttttgatgcccacgattttgccgaccaggcgaaagctggcggcgcaggcgcactactggttagccgtccgctggacatcgacctgccgcagttaatcgtcaaggatacgcgtctggcgtttggtgaactggctgcatgggttcgccagcaagttccggcgcgcgtggttgctctgacggggtcctccggcaaaacctccgttaaagagatgacggcggcgattttaagccagtgcggcaacacgctttatacggcaggcaatctcaacaacgacatcggtgtaccgatgacgctgttgcgcttaacgccggaatacgattacgcagttattgaacttggcgcgaaccatcagggcgaaatagcctggactgtgagtctgactcgcccggaagctgcgctggtcaacaacctggcagcggcgcatctggaaggttttggctcgcttgcgggtgtcgcgaaagcgaaaggtgaaatctttagcggcctgccggaaaacggtatcgccattatgaacgccgacaacaacgactggctgaactggcagagcgtaattggctcacgcaaagtgtggcgtttctcacccaatgccgccaacagcgatttcaccgccaccaatatccatgtgacctcgcacggtacggaatttaccctacaaaccccaaccggtagcgtcgatgttctgctgccgttgccggggcgtcacaatattgcgaatgcgctggcagccgctgcgctctccatgtccgtgggcgcaacgcttgatgctatcaaagcggggctggcaaatctgaaagctgttccaggccgtctgttccccatccaactggcagaaaaccagttgctgctcgacgactcctacaacgccaatgtcggttcaatgactgcagcagtccaggtactggctgaaatgccgggctaccgcgtgctggtggtgggcgatatggcggaactgggcgctgaaagcgaagcctgccatgtacaggtgggcgaggcggcaaaagctgctggtattgaccgcgtgttaagcgtgggtaaacaaagccatgctatcagcaccgccagcggcgttggcgaacattttgctgataaaactgcgttaattacgcgtcttaaatcactgattgctgagcaacaggtaattacgattttagttaagggttcacgtagtgccgccatggaagaggtagtacgcgctttacaggagaatgggacatgttag

SEQ ID NO: 38 - protein, 452 aa, E. coli
MISVTLSQLTDILNGELQGADITLDAVTTDTRKLTPGCLFVALKGERFDAHDFADQAKAGGAGALLVSRPLDIDLPQLIVKDTRLAFGELAAWVRQQVPARVVALTGSSGKTSVKEMTAAILSQCGNTLYTAGNLNNDIGVPMTLLRLTPEYDYAVIELGANHQGEIAWTVSLTRPEAALVNNLAAAHLEGFGSLAGVAKAKGEIFSGLPENGIAIMNADNNDWLNWQSVIGSRKVWRFSPNAANSDFTATNIHVTSHGTEFTLQTPTGSVDVLLPLPGRHNIANALAAAALSMSVGATLDAIKAGLANLKAVPGRLFPIQLAENQLLLDDSYNANVGSMTAAVQVLAEMPGYRVLVVGDMAELGAESEACHVQVGEAAKAAGIDRVLSVGKQSHAISTASGVGEHFADKTALITRLKSLIAEQQVITILVKGSRSAAMEEVVRALQENGTC

SEQ ID NO: 39 - DNA, 642 bp, E. coli
  CDS (1)..(642): E. coli essential gene nadD
atgaaatctttacaggctctgtttggcggcacctttgatccggtgcactatggtcatctaaaacccgtggaaacgctggcgaatttgattggtctgacgcgggtcacaatcatccctaataatgttcctccgcatcgtccccagccggaagcgaacagcgtgcagcgtaaacacatgcttgaactggcgattgccgacaagccattatttactcttgatgaacgcgagctaaagcgcaatgccccctcttacactgcgcaaacactgaaagagtggcggcaggaacaaggaccggacgtgccgctggcgtttattattggtcaggattcattgctgacctttccgacctggtacgaatacgaaacgatactcgacaatgcacatttgatcgtctgtcggcgtccaggttacccacttgaaatggcgcaaccgcaataccagcaatggctggaagatcatttgacacataacccggaagatcttcaccttcagcctgccggtaaaatttatctggctgaaacgccgtggtttaacatctcggcgaccatcatccgcgaacgtttgcaaaacggtgaatcgtgtgaggatttattgccggaaccggtattgacttacattaaccaacaaggcttgtatcgctga

SEQ ID NO: 40 - protein, 213 aa, E. coli
MKSLQALFGGTFDPVHYGHLKPVETLANLIGLTRVTIIPNNVPPHRPQPEANSVQRKHMLELAIADKPLFTLDERELKRNAPSYTAQTLKEWRQEQGPDVPLAFIIGQDSLLTFPTWYEYETILDNAHLIVCRRPGYPLEMAQPQYQQWLEDHLTHNPEDLHLQPAGKIYLAETPWFNISATIIRERLQNGESCEDLLPEPVLTYINQQGLYR

SEQ ID NO: 41 - DNA, 333 bp, E. coli
  CDS (1)..(333): E. coli essential gene rplV
atggaaactatcgctaaacatcgccatgctcgttcttctgctcagaaggttcgccttgttgctgacctgattcgcggtaagaaagtgtcgcaggctctggatattttgacctacaccaacaagaaagcggctgtactggtcaagaaagttctggaatctgccattgctaacgctgaacacaacgatggcgctgacattgacgatctgaaagttacgaaaattttcgtagacgaaggcccgagcatgaagcgcattatgccgcgtgcaaaaggtcgtgcagatcgcatcctgaagcgcaccagccacatcactgtggttgtgtccgatcgctga

SEQ ID NO: 42 - protein, 110 aa, E. coli [sequence omitted]

SEQ ID NO: 43 - DNA, 471 bp, E. coli
  CDS (1)..(471): E. coli essential gene rpsG
atgccacgtcgtcgcgtcattggtcagcgtaaaattctgccggatccgaagttcggatcagaactgctggctaaatttgtaaatatcctgatggtagatggtaaaaaatctactgctgaatctatcgtatacagcgcgctggagaccctggctcagcgctctggtaaatctgaactggaagcattcgaagtagctctcgaaaacgtgcgcccgactgtagaagttaagtctcgccgcgttggtggttctacttatcaggtaccagttgaagtccgtccggttcgtcgtaatgctctggcaatgcgttggatcgttgaagctgctcgtaaacgcggtgataaatccatggctctgcgcctggcgaacgaactttctgatgctgcagaaaacaaaggtactgcagttaagaaacgtgaagacgttcaccgtatggccgaagccaacaaggcgttcgcacactaccgttggtaa

SEQ ID NO: 44 - protein, 156 aa, E. coli
MPRRRVIGQRKILPDPKFGSELLAKFVNILMVDGKKSTAESIVYSALETLAQRSGKSELEAFEVALENVRPTVEVKSRRVGGSTYQVPVEVRPVRRNALAMRWIVEAARKRGDKSMALRLANELSDAAENKGTAVKKREDVHRMAEANKAFAHYRW

SEQ ID NO: 45 - DNA, 2475 bp, S. cerevisiae
  CDS (1)..(2475): S. cerevisiae essential gene FOL1 YNL256W SGDID:S000005200
atgtcaaagctattttctactgtcaattctgcaagacatagtgtaccactaggcggcatgagagattatgtgcacattaagaaactagagatgaatacagttcttgggcctgattcctggaatcaattaatgcctcagaaatgtctactaagcttagatatgggtacagattttagtaaatctgcggctacggatgatttgaaatattctctaaattatgcagttatttctcgtgatttgacgaatttcgtcagcaaaaaaaagaattggggttctgtttctaatttggctaaatctgtgtctcaatttgttatggacaaatattctggtgtcgagtgtctgaatttagaagtgcaggcggatacaacgcatattagaagtgaccacatatcttgtattattcaacaagaaagagggaatccagaatcacaggaatttgacgttgttaggatatctgagttaaaaatgttgactttgattggtgttttcacctttgagagacttaagaaacagtatgtaactttggatataaagttgccttggccaaagaaagccgaattgccaccgccagtgcaaagcataattgataacgttgtcaagtttgtggaggaatcaaatttcaagactgtggaagctcttgtagaatctgtgtcagctgttattgcccataacgagtattttcaaaagtttccagattcgcctttggtggtgaaggttttgaaattaaacgcaatcacagccacagaaggtgttggtgtaagctgtattagagagcccagggagattgcgatggtaaatattccatatctttcctccatacatgaatcgtctgatattaagttccaattgtcttcatcacaaaacactcctattgagggtaaaaatacatggaaaagagcgtttttagcgtttggttcaaacattggggaccgtttcaaacacattcaaatggcgttgcaattattatcaagggaaaaaacggttaaattacggaatatttcgtctatttttgaaagtgaaccaatgtatttcaaagatcaaacccctttcatgaatgggtgtgttgaggtggagacattactgaccccaagcgaattattaaaattgtgtaaaaaaattgaatatgaagagttgcaaagagtcaagcattttgataatggtccgagaacaatagatctggatattgttatgtttttgaatagcgccggagaagatattatagtaaatgaaccggatttgaatataccgcatcctagaatgctggagaggactttcgttcttgagccgttatgtgaattaatatcccccgttcaccttcatcctgtgacagcggaacccattgtagaccatttaaaacagttatacgacaaacagcatgatgaagataccttatggaaattagttccattgccttatcgtagtggtgtggagcctagatttttgaaattcaagaccgctacaaaacttgacgaatttactggagaaacaaacagaattactgtttcacctacatatatcatggctatcttcaacgctacaccagattcattttccgatggaggtgagcattttgcggacattgaaagtcaattgaatgatatcattaaattgtgtaaagacgcattatatttgcatgagagcgtcatcatcgacgttggagggtgttctaccaggcctaactctattcaggcgtctgaggaagaagaaatacgcaggtctatcccattaattaaggccattagagaaagcactgagttaccgcaagataaagtcatactatccattgatacttatcgttccaatgtcgctaaagaagcgattaaagttggagtggatattattaatgatatttcgggaggtttatttgacagcaacatgtttgccgtaattgcagagaacccagaaatttgttatattttatcacacacacgtggtgatatttcaacgatgaataggctggcgcattacgaaaattttgcattgggtgattctattcagcaagaatttgttcataataccgacattcagcagctagacgacttgaaagacaaaacagtgttaatcaggaatgttggtcaagaaattggcgaaaggtatatcaaagcgattgataatggagtaaagcgctggcaaattctaatcgaccctggacttggttttgctaagacctggaagcaaaacttacaaattattagacatatccccattttaaagaactactcattcaccatgaactcaaacaattcgcaagtgtatgttaacctcagaaatatgcccgttttattgggtccatcgcgcaaaaaattcattggacatatcacaaaagatgtggatgcgaagcaaagagactttgctactggagcggtggtagcgtcgtgtattggtttcggcagcgacatggttagggtccatgacgttaaaaattgttcgaagagcattaaattagcagatgctatttataaaggtttggaataa

SEQ ID NO: 46 - protein, 824 aa, S. cerevisiae
MSKLFSTVNSARHSVPLGGMRDYVHIKKLEMNTVLGPDSWNQLMPQKCLLSLDMGTDFSKSAATDDLKYSLNYAVISRDLTNFVSKKKNWGSVSNLAKSVSQFVMDKYSGVECLNLEVQADTTHIRSDHISCIIQQERGNPESQEFDVVRISELKMLTLIGVFTFERLKKQYVTLDIKLPWPKKAELPPPVQSIIDNVVKFVEESNFKTVEALVESVSAVIAHNEYFQKFPDSPLVVKVLKLNAITATEGVGVSCIREPREIAMVNIPYLSSIHESSDIKFQLSSSQNTPIEGKNTWKRAFLAFGSNIGDRFKHIQMALQLLSREKTVKLRNISSIFESEPMYFKDQTPFMNGCVEVETLLTPSELLKLCKKIEYEELQRVKHFDNGPRTIDLDIVMFLNSAGEDIIVNEPDLNIPHPRMLERTFVLEPLCELISPVHLHPVTAEPIVDHLKQLYDKQHDEDTLWKLVPLPYRSGVEPRFLKFKTATKLDEFTGETNRITVSPTYIMAIFNATPDSFSDGGEHFADIESQLNDIIKLCKDALYLHESVIIDVGGCSTRPNSIQASEEEEIRRSIPLIKAIRESTELPQDKVILSIDTYRSNVAKEAIKVGVDIINDISGGLFDSNMFAVIAENPEICYILSHTRGDISTMNRLAHYENFALGDSIQQEFVHNTDIQQLDDLKDKTVLIRNVGQEIGERYIKAIDNGVKRWQILIDPGLGFAKTWKQNLQIIRHIPILKNYSFTMNSNNSQVYVNLRNMPVLLGPSRKKFIGHITKDVDAKQRDFATGAVVASCIGFGSDMVRVHDVKNCSKSIKLADAIYKGLE

SEQ ID NO: 47 - DNA, 669 bp, S. cerevisiae
  CDS (1)..(669): S. cerevisiae essential gene MED7 YOL135C SGDID:S000005495
atgtccaatgatcctggtaatgaggttagctccttgtacccacctccacccccatacgtgaagtttttcacacagtccaatctggaaaaattaccaaaatacaaagaaaagaaggccgcaagtgcgaagcagacggctccaaataacagtaacggcggcagtgaagaggagattacatgtgcgctagattacctaatcccaccccccatgcccaaaaatcagcagtaccgagcgtttgggagtatatggcaggtgaaggaccaactgcccgatttagagagcatgggactcacccaactttataagaaatccacagaaaacgaaagcacaaattatcaatacaaaatccaagagctacgcaaactattgaaatccctcctgctaaattacttggaactcatcggcgtattgagcataaatccggatatgtatgagcgcaaagtggagaacataaggaccattcttgtcaatattcaccacctacttaatgagtacagaccccatcagtcccgagagtcccttattatgctattggaagaacaattagaatacaagcgcggggaaattcgcgagatcgagcaagtatgcaaacaggtacacgacaaactcaccagcatacaggacaccttaagaaccggatcacaatctcctccatcgtcgtcccaatga

SEQ ID NO: 48 - protein, 222 aa, S. cerevisiae
MSNDPGNEVSSLYPPPPPYVKFFTQSNLEKLPKYKEKKAASAKQTAPNNSNGGSEEEITCALDYLIPPPMPKNQQYRAFGSIWQVKDQLPDLESMGLTQLYKKSTENESTNYQYKIQELRKLLKSLLLNYLELIGVLSINPDMYERKVENIRTILVNIHHLLNEYRPHQSRESLIMLLEEQLEYKRGEIREIEQVCKQVHDKLTSIQDTLRTGSQSPPSSSQ

SEQ ID NO: 49 - DNA, 723 bp, S. cerevisiae
  CDS (1)..(723): S. cerevisiae essential gene RRP40 YOL142W SGDID:S000005502
atgtctacgttcatattccctggtgatagctttcctgtagaccctactacacctgttaaactgggccctggcatatattgtgaccccaatactcaagaaatacgacctgttaatacaggtgttttgcatgtttccgctaagggtaagagtggtgttcagaccgcatatatagactattctagtaagagatacattccatctgtaaacgattttgtaatcggtgtcattatagggacattttcagatagctataaggtttcgttgcaaaatttctcctccagtgtttcactatcgtatatggcttttcccaatgcttcaaagaaaaacaggccaactttgcaagtgggagatctagtgtatgcgagagtttgtaccgcagaaaaggaactagaagccgaaatagaatgttttgactcaactacaggacgcgatgctggtttcgggatattggaagatggtatgatcattgacgtgaatttgaatttcgcacgccagttgcttttcaataatgacttcccgttattaaaagtgttggctgcacataccaagtttgaagtcgccattggtctcaatgggaagatctgggttaagtgcgaggaattatctaacactttagcttgttatagaaccataatggagtgttgtcaaaaaaacgacacggcagcgttcaaggatatagcaaaaagacagtttaaagaaatacttacggtcaaggaggagtag

SEQ ID NO: 50 - protein, 240 aa, S. cerevisiae
MSTFIFPGDSFPVDPTTPVKLGPGIYCDPNTQEIRPVNTGVLHVSAKGKSGVQTAYIDYSSKRYIPSVNDFVIGVIIGTFSDSYKVSLQNFSSSVSLSYMAFPNASKKNRPTLQVGDLVYARVCTAEKELEAEIECFDSTTGRDAGFGILEDGMIIDVNLNFARQLLFNNDFPLLKVLAAHTKFEVAIGLNGKIWVKCEELSNTLACYRTIMECCQKNDTAAFKDIAKRQFKEILTVKEE

SEQ ID NO: 51 - DNA, 1455 bp, S. cerevisiea
  CDS (1)..(1455): S. cerevisiae essential gene NOP8 YOL144W SGDID:S000005504
atggatagtgtaattcaaaaaagaatttttgtcggaaatattttccataatgcagatgattgttattcagaactactagatcgatttggaaaatttggtgattgccaagattttcagtttgaaaaacacaaccactttgcatttatcgatataaggtttaatgatgaggcagattttaacaagctaagaaagagctttaataatgttaagtttaaagggaacattttgaaggttgatgaagcaaagccgaattgggaaagcacctgggcggtacaacatgcaaaggaccttaaagaagatattatactaaatgctaaaatgaaaaaaaagaattggcaacattataagaaaatggaaaatgtagcgaaaagttggaaagatcataaggaagttattgctggcagaatgagggaggcgccgagaaaaaggagtcaattgaggaacattacattcaggatcaatgtcaatggttcattgaaagtttacaaatgctataagactaaattatggggttatgaaaggaacaaagaattgaatgaccttgtgtacaagtttacaaataatttctggaaaaacggatacaaccacattgtcgatagattggattacagtcgtgctgttaaaactgttcgattcaaaaatgggctgaaacagttaacagtgtcaaaagatgaaaacgtttgcagtggagagatggacagcgatgagaatatgtcagaagaggagaaggagaaaaataatgttattcttaatgacctattaaaggactttgacttcgataagccaatgacgttgaatgattcggacgaggaacttctgacagagcaacgtaaaggagaggaagaagaagaagaagaagaagaaaaagaagtaaacgctcccgaatacgagaatgttaataagacgaaggaccagagcaccctaccacaagaaaaaccagaggaaaggaaagaacaggacgagggcgacgggcaggaggataatgaatttattccgactttcaccaaggaaattggtcaaggtacaataagcaacactgagacgttaagaaacctattcaaccccaacgaggcagaacctgtatcacaattcaaattgattgaagattctgataatgatattgatcatgcgaaagatgttgatgtgaaccaactggaggaagaagtaagtaaatcatctgacaccctaggtttgacatcggctcccgtaccacatgtatctagagataaagataacaaaaatttcttgtttttccctcatttgcaatcgccatttttagtaggacaaacacagttgagtaaagtaagggctcctggaagagaaacaatgctatcgaactgggatgaggagttctgggctaacagaggtaattggacccgtgatatgaggcgcaaaatgaaagatgcattgaagcaccgtaagaggaaacaatcaaagagcgggcttcttctatag

SEQ ID NO: 52 - protein, 484 aa, S. cerevisiea
MDSVIQKRIFVGNIFHNADDCYSELLDRFGKFGDCQDFQFEKHNHFAFIDIRFNDEADFNKLRKSFNNVKFKGNILKVDEAKPNWESTWAVQHAKDLKEDIILNAKMKKKNWQHYKKMENVAKSWKDHKEVIAGRMREAPRKRSQLRNITFRINVNGSLKVYKCYKTKLWGYERNKELNDLVYKFTNNFWKNGYNHIVDRLDYSRAVKTVRFKNGLKQLTVSKDENVCSGEMDSDENMSEEEKEKNNVILNDLLKDFDFDKPMTLNDSDEELLTEQRKGEEEEEEEEEKEVNAPEYENVNKTKDQSTLPQEKPEERKEQDEGDGQEDNEFIPTFTKEIGQGTISNTETLRNLFNPNEAEPVSQFKLIEDSDNDIDHAKDVDVNQLEEEVSKSSDTLGLTSAPVPHVSRDKDNKNFLFFPHLQSPFLVGQTQLSKVRAPGRETMLSNWDEEFWANRGNWTRDMRRKMKDALKHRKRKQSKSGLLL

SEQ ID NO: 53 - DNA, 1665 bp, S. cerevisiae
  CDS (1)..(1665): S. cerevisiae essential gene PGI1 YBR196C SGDID:S000000400
atgtccaataactcattcactaacttcaaactggccactgaattgccagcctggtctaagttgcaaaaaatttatgaatctcaaggtaagactttgtctgtcaagcaagaattccaaaaagatgccaagcgttttgaaaaattgaacaagactttcaccaactatgatggttccaaaatcttgttcgactactcaaagaacttggtcaacgatgaaatcattgctgcattgattgaactggccaaggaggctaacgtcaccggtttgagagatgctatgttcaaaggtgaacacatcaactccactgaagatcgtgctgtctaccacgtcgcattgagaaacagagctaacaagccaatgtacgttgatggtgtcaacgttgctccagaagtcgactctgtcttgaagcacatgaaggagttctctgaacaagttcgttctggtgaatggaagggttataccggtaagaagatcaccgatgttgttaacatcggtattggtggttccgatttgggtccagtcatggtcactgaggctttgaagcactacgctggtgtcttggatgtccacttcgtttccaacattgacggtactcacattgctgaaaccttgaaggttgttgacccagaaactactttgtttttgattgcttccaagactttcactaccgctgaaactatcactaacgctaacactgccaagaactggttcttgtcgaagacaggtaatgatccatctcacattgctaagcatttcgctgctttgtccactaacgaaaccgaagttgccaagttcggtattgacaccaaaaacatgtttggtttcgaaagttgggtcggtggtcgttactctgtctggtcggctattggtttgtctgttgccttgtacattggctatgacaactttgaggctttcttgaagggtgctgaagccgtcgacaaccacttcacccaaaccccattggaagacaacattccattgttgggtggtttgttgtctgtctggtacaacaacttctttggtgctcaaacccatttggttgctccattcgaccaatacttgcacagattcccagcctacttgcaacaattgtcaatggaatctaacggtaagtctgttaccagaggtaacgtgtttactgactactctactggttctatcttgtttggtgaaccagctaccaacgctcaacactctttcttccaattggttcaccaaggtaccaagttgattccatctgatttcatcttagctgctcaatctcataacccaattgagaacaaattacatcaaaagatgttggcttcaaacttctttgctcaagctgaagctttaatggttggtaaggatgaagaacaagttaaggctgaaggtgccactggtggtttggtcccacacaaggtcttctcaggtaacagaccaactacctctatcttggctcaaaagattactccagctactttgggtgctttgattgcctactacgaacatgttactttcactgaaggtgccatttggaatatcaactctttcgaccaatggggtgttgaattgggtaaagtcttggctaaagtcatcggcaaggaattggacaactcctccaccatttctacccacgatgcttctaccaacggtttaatcaatcaattcaaggaatggatgtga

SEQ ID NO: 54 - protein, 554 aa, S. cerevisiae
MSNNSFTNFKLATELPAWSKLQKIYESQGKTLSVKQEFQKDAKRFEKLNKTFTNYDGSKILFDYSKNLVNDEIIAALIELAKEANVTGLRDAMFKGEHINSTEDRAVYHVALRNRANKPMYVDGVNVAPEVDSVLKHMKEFSEQVRSGEWKGYTGKKITDVVNIGIGGSDLGPVMVTEALKHYAGVLDVHFVSNIDGTHIAETLKVVDPETTLFLIASKTFTTAETITNANTAKNWFLSKTGNDPSHIAKHFAALSTNETEVAKFGIDTKNMFGFESWVGGRYSVWSAIGLSVALYIGYDNFEAFLKGAEAVDNHFTQTPLEDNIPLLGGLLSVWYNNFFGAQTHLVAPFDQYLHRFPAYLQQLSMESNGKSVTRGNVFTDYSTGSILFGEPATNAQHSFFQLVHQGTKLIPSDFILAAQSHNPIENKLHQKMLASNFFAQAEALMVGKDEEQVKAEGATGGLVPHKVFSGNRPTTSILAQKITPATLGALIAYYEHVTFTEGAIWNINSFDQWGVELGKVLAKVIGKELDNSSTISTHDASTNGLINQFKEWM

SEQ ID NO: 55 - DNA, 759 bp, S. cerevisiae
  CDS (1)..(759): S. cerevisiae essential gene NEP1 EMG1 YLR186W SGDID:S000004176
atggtcgaagattccagagttagagacgccctcaaaggtggtgatcagaaggcattaccggcctctttggttcctcaagcacctcctgtcttgacatcaaaggataagattactaagcggatgattgtggtattagcgatggcatccctcgagacacacaagatatcgtccaacgggcctggtggtgacaaatatgtccttttgaactgtgacgaccatcaaggtttattaaaaaaaatgggtagagacattagtgaagcaagacctgatattacccaccaatgtcttttgacgttgctagattctccaatcaacaaagccggaaagctgcaggtctatattcaaacaagtcgaggaattctgatcgaggttaaccccactgttcgtataccaagaactttcaaaagattttcaggtttaatggttcagttactacataagctttctatcagatcggtaaattctgaagaaaagttacttaaagtcattaagaacccaattaccgatcacctacctactaagtgccgtaaggtgacattatcctttgacgcaccagttatccgcgttcaagattacatcgaaaaactagacgatgatgaaagtatatgtgtctttgttggtgccatggcaagaggtaaagataactttgcggatgaatacgtcgacgaaaaagtcggcttgtccaattacccattgtctgcctcagttgcatgttctaaattttgccatggcgctgaagatgcttggaatattttatag

SEQ ID NO: 56 - protein, 252 aa, S. cerevisiae
MVEDSRVRDALKGGDQKALPASLVPQAPPVLTSKDKITKRMIVVLAMASLETHKISSNGPGGDKYVLLNCDDHQGLLKKMGRDISEARPDITHQCLLTLLDSPINKAGKLQVYIQTSRGILIEVNPTVRIPRTFKRFSGLMVQLLHKLSIRSVNSEEKLLKVIKNPITDHLPTKCRKVTLSFDAPVIRVQDYIEKLDDDESICVFVGAMARGKDNFADEYVDEKVGLSNYPLSASVACSKFCHGAEDAWNIL

SEQ ID NO: 57 - DNA, 804 bp, S. cerevisiea
  CDS (1)..(804): S. cerevisea essential gene URA3
atgtcgaaagctacatataaggaacgtgctgctactcatcctagtcctgttgctgccaagctatttaatatcatgcacgaaaagcaaacaaacttgtgtgcttcattggatgttcgtaccaccaaggaattactggagttagttgaagcattaggtcccaaaatttgtttactaaaaacacatgtggatatcttgactgatttttccatggagggcacagttaagccgctaaaggcattatccgccaagtacaattttttactcttcgaagacagaaaatttgctgacattggtaatacagtcaaattgcagtactctgcgggtgtatacagaatagcagaatgggcagacattacgaatgcacacggtgtggtgggcccaggtattgttagcggtttgaagcaggcggcagaagaagtaacaaaggaacctagaggccttttgatgttagcagaattgtcatgcaagggctccctatctactggagaatatactaagggtactgttgacattgcgaagagcgacaaagattttgttatcggctttattgctcaaagagacatgggtggaagagatgaaggttacgattggttgattatgacacccggtgtgggtttagatgacaagggagacgcattgggtcaacagtatagaaccgtggatgatgtggtctctacaggatctgacattattattgttggaagaggactatttgcaaagggaagggatgctaaggtagagggtgaacgttacagaaaagcaggctgggaagcatatttgagaagatgcggccagcaaaactaa

SEQ ID NO: 58 - protein, 267 aa, S. cerevisiea
MSKATYKERAATHPSPVAAKLFNIMHEKQTNLCASLDVRTTKELLELVEALGPKICLLKTHVDILTDFSMEGTVKPLKALSAKYNFLLFEDRKFADIGNTVKLQYSAGVYRIAEWADITNAHGVVGPGIVSGLKQAAEEVTKEPRGLLMLAELSCKGSLSTGEYTKGTVDIAKSDKDFVIGFIAQRDMGGRDEGYDWLIMTPGVGLDDKGDALGQQYRTVDDVVSTGSDIIIVGRGLFAKGRDAKVEGERYRKAGWEAYLRRCGQQN

SEQ ID NO: 59 - DNA, 1095 bp, S. cerevisiae
  CDS (1)..(1095): S. ceverisiae essential gene LEU2
atgtctgcccctaagaagatcgtcgttttgccaggtgaccacgttggtcaagaaatcacagccgaagccattaaggttcttaaagctatttctgatgttcgttccaatgtcaagttcgatttcgaaaatcatttaattggtggtgctgctatcgatgctacaggtgtcccacttccagatgaggcgctggaagcctccaagaaggttgatgccgttttgttaggtgctgtggctggtcctaaatggggtaccggtagtgttagacctgaacaaggtttactaaaaatccgtaaagaacttcaattgtacgccaacttaagaccatgtaactttgcatccgactctcttttagacttatctccaatcaagccacaatttgctaaaggtactgacttcgttgttgtcagagaattagtgggaggtatttactttggtaagagaaaggaagacgatggtgatggtgtcgcttgggatagtgaacaatacaccgttccagaagtgcaaagaatcacaagaatggccgctttcatggccctacaacatgagccaccattgcctatttggtccttggataaagctaatcttttggcctcttcaagattatggagaaaaactgtggaggaaaccatcaagaacgaattccctacattgaaggttcaacatcaattgattgattctgccgccatgatcctagttaagaacccaacccacctaaatggtattataatcaccagcaacatgtttggtgatatcatctccgatgaagcctccgttatcccaggttccttgggtttgttgccatctgcgtccttggcctctttgccagacaagaacaccgcatttggtttgtacgaaccatgccacggttctgctccagatttgccaaagaataaggttgaccctatcgccactatcttgtctgctgcaatgatgttgaaattgtcattgaacttgcctgaagaaggtaaggccattgaagatgcagttaaaaaggttttggatgcaggtatcagaactggtgatttaggtggttccaacagtaccaccgaagtcggtgatgctgtcgccgaagaagttaagaaaatccttgcttaa

SEQ ID NO: 60 - protein, 364 aa, S. cerevisiae
MSAPKKIVVLPGDHVGQEITAEAIKVLKAISDVRSNVKFDFENHLIGGAAIDATGVPLPDEALEASKKVDAVLLGAVAGPKWGTGSVRPEQGLLKIRKELQLYANLRPCNFASDSLLDLSPIKPQFAKGTDFVVVRELVGGIYFGKRKEDDGDGVAWDSEQYTVPEVQRITRMAAFMALQHEPPLPIWSLDKANLLASSRLWRKTVEETIKNEFPTLKVQHQLIDSAAMILVKNPTHLNGIIITSNMFGDIISDEASVIPGSLGLLPSASLASLPDKNTAFGLYEPCHGSAPDLPKNKVDPIATILSAAMMLKLSLNLPEEGKAIEDAVKKVLDAGIRTGDLGGSNSTTEVGDAVAEEVKKILA

SEQ ID NO: 61 - DNA, 675 bp, S. cerevisiae
  CDS (1)..(675): S. cerevisiae essential gene TRP1
atgtctgttattaatttcacaggtagttctggtccattggtgaaagtttgcggcttgcagagcacagaggccgcagaatgtgctctagattccgatgctgacttgctgggtattatatgtgtgcccaatagaaagagaacaattgacccggttattgcaaggaaaatttcaagtcttgtaaaagcatataaaaatagttcaggcactccgaaatacttggttggcgtgtttcgtaatcaacctaaggaggatgttttggctctggtcaatgattacggcattgatatcgtccaactgcatggagatgagtcgtggcaagaataccaagagttcctcggtttgccagttattaaaagactcgtatttccaaaagactgcaacatactactcagtgcagcttcacagaaacctcattcgtttattcccttgtttgattcagaagcaggtgggacaggtgaacttttggattggaactcgatttctgactgggttggaaggcaagagagccccgaaagcttacattttatgttagctggtggactgacgccagaaaatgttggtgatgcgcttagattaaatggcgttattggtgttgatgtaagcggaggtgtggagacaaatggtgtaaaagactctaacaaaatagcaaatttcgtcaaaaatgctaagaaatag

SEQ ID NO: 62 - protein, 224 aa, S. cerevisiae
MSVINFTGSSGPLVKVCGLQSTEAAECALDSDADLLGIICVPNRKRTIDPVIARKISSLVKAYKNSSGTPKYLVGVFRNQPKEDVLALVNDYGIDIVQLHGDESWQEYQEFLGLPVIKRLVFPKDCNILLSAASQKPHSFIPLFDSEAGGTGELLDWNSISDWVGRQESPESLHFMLAGGLTPENVGDALRLNGVIGVDVSGGVETNGVKDSNKIANFVKNAKK

SEQ ID NO: 63 - DNA, 657 bp, S. cerevisiae
  CDS (1)..(657): S. cerevisiae essential gene HIS3
atgacagagcagaaagccctagtaaagcgtattacaaatgaaaccaagattcagattgcgatctctttaaagggtggtcccctagcgatagagcactcgatcttcccagaaaaagaggcagaagcagtagcagaacaggccacacaatcgcaagtgattaacgtccacacaggtatagggtttctggaccatatgatacatgctctggccaagcattccggctggtcgctaatcgttgagtgcattggtgacttacacatagacgaccatcacaccactgaagactgcgggattgctctcggtcaagcttttaaagaggccctactggcgcgtggagtaaaaaggtttggatcaggatttgcgcctttggatgaggcactttccagagcggtggtagatctttcgaacaggccgtacgcagttgtcgaacttggtttgcaaagggagaaagtaggagatctctcttgcgagatgatcccgcattttcttgaaagctttgcagaggctagcagaattaccctccacgttgattgtctgcgaggcaagaatgatcatcaccgtagtgagagtgcgttcaaggctcttgcggttgccataagagaagccacctcgcccaatggtaccaacgatgttccctccaccaaaggtgttcttatg

SEQ ID NO: 64 - protein, 219 aa, S. cerevisiae
MTEQKALVKRITNETKIQIAISLKGGPLAIEHSIFPEKEAEAVAEQATQSQVINVHTGIGFLDHMIHALAKHSGWSLIVECIGDLHIDDHHTTEDCGIALGQAFKEALLARGVKRFGSGFAPLDEALSRAVVDLSNRPYAVVELGLQREKVGDLSCEMIPHFLESFAEASRITLHVDCLRGKNDHHRSESAFKALAVAIREATSPNGTNDVPSTKGVLM

SEQ ID NO: 65 - DNA, 290 bp, E. coli
  promoter (1)..(290): burden sensing promoter p(htpG)
gccaccaaccccacggttgaaggtgaagctaccgctaactacattgccgagctttgcgcgcaatatgacgtggaagccagccgaatcgctcatggcgtaccggttggcggcgaactggaaatggtcgatggcaccacgctgtcacactcccttgccgggcgtcataagattcgtttttaagcaaacgagagcaggatcacctgctctcgcttgaaattattctcccttgtccccatctctccctcatcctgtttttaaccttaaaatggcattattgaggtagacctaca

SEQ ID NO: 66 - DNA, 257 bp, E. coli
  promoter (1)..(257): burden sensing promoter p(ibpA)
atcccttgctgaaaataacatcatcattacgtcgcactgtggcggctatcgcactttaacgtttcgtgctgccccctcagtctatgcaatagaccataaactgcaaaaaaaagtccgctgataaggcttgaaaagttcatttccagacccatttttacatcgtagccgatgaggacgcgcctgatgggtgttctggctacctgacctgtccattgtggaaggtcttacattctcgctgatttcaggagctattgatt

SEQ ID NO: 67 - DNA, 298 bp, E.coli
  promoter (1)..(298): burden sensing promoter p(clpB)
gataagtatctggcggatatttatctgcttgcccggcagcgtctggcgagcgttggtgttgaacaaattttcggcggcgaccgttgtacatatacggaaaatgagactttcttctcttatcgtcgcgacaagaccaccgggcgtatggcaagtttcatttggctgatataacctaaagaatcaagacgatccggtacgcgtgattttcttttcacattaatctggtcaataaccttgaataattgagggatgacctcatttaatctccagtagcaactttgatccgttatgggaggag

SEQ ID NO: 68 - DNA, 300 bp, E. coli
  promoter (1)..(300): burden sensing promoter p(yccV)
ggttataaagacatcaacatgctggcgattcagctgctgaatgaaggcggtattctcctgactttctcctgttccggtctgatgaccagcgatttatttcagaaaatcatcgcggatgccgcaattgatgccggtcgtgatgtacaatttatagagcagttccgtcaggcagccgatcatccggtgatcgctacctatccggaagggctatatctgaaagggtttgcctgtcgcgtcatgtaacttgaaatgtggaattttacccttatatcaaaggtaaagatttcccgggaggtgact

SEQ ID NO: 69 - DNA, 300 bp, E. coli
  promoter (1)..(300): burden sensing promoter p(grpE)
tctccgcgagcgtgccagttttcacattcttcagttgcagttcgtgagcgatttgttgctcaacgatgacctcgtaaccttttgtgcacagccagcggtagagcatttcatgtgttgtcagtgcagtggggtgccgtgggtgtcccacaatgccaatacacttgaaatgattattcatttttccgaggtccttgttgcgaagattgatgacaatgtgagtgcttcccttgaaaccctgaaactgatccccataataagcgaagttagcgagatgaatgcgaaaaaaacgcggagaaattc

SEQ ID NO: 70 - DNA, 300 bp, E. coli
  promoter (1)..(300): burden sensing promoter p(ycjX)
ttggctgatactgtaattcttcaatggcccgtaacactttttcgcgcgcttccggggagatattagtttgcttattcagcacgcgtgatacggtggattttgatacgcctgcaaccctggcaatatcataaatagtaggggacataggtcaggaactccgtccgaacgtgaatgctgcacatcttatggagttcgccggtcgatgacaacacgggcagttgataatcaatggcctggcccccacattcatatccttacgaatgattttttttctggtcttcagagcagcacaggacagca

SEQ ID NO: 71 - DNA, 300 bp, E. coli
  promoter (1)..(300): burden sensing promoter p(ldhA)
gggaacccacagcccgagcgtcatcagcagcgtcaacggcacaagaataatcagtaataacagcgcgagaacggctttatatttacccagcatgggtagttaatatcctgatttagcgaaaaattaagcattcaatacgggtattgtggcatgtttaaccgttcagttgaaggttgcgcctacactaagcatagttgttgatgaatttttcaatatcgccatagctttcaattatatttgaaattttgtaaaatatttttagtagcttaaatgtgattcaacatcactggagaaagtctt

SEQ ID NO: 72 - DNA, 300 bp, E. coli
  promoter (1)..(300): burden sensing promoter p(mutM)
ggcgaaaagtactaagtacttagaggaaataaatcatggctaaaggtattcgtgagaaaatcaagctggtttcttctgctggtactggtcacttctataccactacgaagaacaaacgtactaagccggaaaaactggaactgaaaaaattcgatccagttgttcgccagcacgtgatctacaaagaagcgaaaatcaaataattctcgctttgatgtaacaaaaaacctcgctccggcggggttttttgttatctgcttgcccccatattgactgcatctgttcattcctggagatgct

SEQ ID NO: 73 - DNA, 300 bp, E. coli
  promoter (1)..(300): burden sensing promoter p(ybbN)
cccattcgtactcgcttcaccgacaacgtcaaccagacgcaaagtgataaaccagtcgaaaatcccggcatcgccgcccgctttacgttgggaccggaagcggtggtggacaaagtacgccatgcttttattagcgagaagccgaagatgcgctatccggtaacgctggtgacctgggcagtaatggtgcttaagcgcctgctgccggggcgcgtgatggacaaaatattgcaggggtgagttgaagcgcgcgcttaagcccccatgtcaaagaaaatatcgacaacagagagcgactcc

SEQ ID NO: 74 - DNA, 298 bp, E. coli
  promoter (1)..(298): burden sensing promoter p(prlC)
agttcttgtttgagtccactcatgggttgatgtccgattgcgcccaaattttgggcaactgcgtagattttcgatggtagcacaatcagattcgcttatgacggtgatgaagaaattgcgatgaaatgtgaggtgaatcagggttttcacccgattttgtgctgatcagaattttttttctttttcccccttgaaggggcgaagcctcatccccatttctctggtcaccagccgggaaaccacgtaagctccggcgtcacccataacagatacggactttctcaaaggagagttatca

SEQ ID NO: 75 - DNA, 298 bp, E. coli; identical to SEQ ID NO: 74
  promoter (1)..(298): burden sensing promoter p(groES)

SEQ ID NO: 76 - DNA, 392 bp, E. coli
  promoter (1)..(392): burden sensing promoter p(fxsA)
  misc_feature (328)..(328): n is a, c, g, or t
gatccccggaatattcatatgttaaacacacagaatatatgtggtttcgaatgtttttcgaccgacgattatcccctgcatcgaccgaatacccgagatcatatgctgcttgaggatttctaccgtaatctggatcactttaagtgtcggtttttaccccttaattattaatttgtgaaatagatcaccgctttgggattactaccaaaaatagttgcgcaaacatcttgaaattttgctaatgaccacaatataagctgaacgcgattcgcaacccattcaggtagccgggttttaccggctgctattacaggagaaacctacttgnaaggtatgaaactctttgcccagggtacttcactggaccttagccatcctcacgtaatggggat

SEQ ID NO: 77 - DNA, 300 bp, E. coli
  promoter (1)..(300): burden sensing promoter p(htpX)
agattaccaggagccggatccttatctggatgagacggtgaatatcgcactcgatctggcgaagcttgaaaaagccagacccgcggaacaacccgctcccgtcaagtaatatcaatcaggcacaagaaattgtgcctgattttttaacagcggcaagatgccgtaaatcagatgctacaaaatgtaaagttgtgtctttctggtgacttacgcactatccagacttgaaaatagtcgcgtaacccatacgatgtgggtatcgcatattgcgttttgttaaactgaggtaaaaagaaaatt

SEQ ID NO: 78 - DNA, 275 bp, E. coli
  promoter (1)..(275): burden sensing promoter p(rrnB)
gcaaacacgccgccgggtcagcggggttctcctgagaattccggcagagaaagcaaaaataaatgcttgactctgtagcgggaaagcgtattatgcacaccccgcgccgctgagaaaaagcgaagcggcactgctctttaacaatttatcagacaatctgtgtgggcactcgaagatacggattcttaacgtcgcaagacgaaaaatgaataccaagtctcaagagtgaacacgtaattcattacgaagtttaattctttgagcgtcaaactttt

SEQ ID NO: 79 - DNA, 296 bp, E. coli
  promoter (1)..(296): burden sensing promoter p(rrnE)
aatgcgcctccgttgagacgacaacgtgaaacacttcacaggatggtcggaacaacgaagagaaaaaaatcctgaaattcagggttgactctgaaagaggaaagcgtaatatacgccacctcgcgacagtgagctgaaagccgcgtcgcaactgctctttaacaatttatcagacaatctgtgtgggcactcgaagatacggattcttaacgtcgcaagacgaaaaatgaataccaagtctcaagagtgaacacgtaattcattacgaagtttaattctttgagcatcaaactttt

SEQ ID NO: 80 - DNA, 300 bp, E. coli
  promoter (1)..(300): burden sensing promoter p(cspD)
cggttatcggcagaacgccctgccgctgacaagagcttatttgcctgaccaatctactccacatgatagataactatcatctatcgttggcatcagcgacatctgtcacattcctgtcaatagcgttaactgcttcaaatttttgattcatacctgccccctgtcccctgtcaaatgcttgacggctcgccctaattctctaaattgtatttctagagttggcgaggttttgaacagccccctctctgaccccggtttattccatcttacttgtataagatttgcgaaggatgtcgaagc

SEQ ID NO: 81 - DNA, 299 bp, E. coli
  promoter (1)..(299): burden sensing promoter p(katE)
taaatccatctttatcgcatgttctggcggcgcgggttccgtgcgtgggacatagctaataatctggcggttttgctggcggagcggtttcttcattactggcttcactaaacgcatattaaaaatcagaaaaactgtagtttagccgatttagcccctgtacgtcccgctttgcgtgtatttcataacaccgtttccagaatagtctccgaagcgggatctggctggtggtctatagttagagagttttttgaccaaaacagcggccctttcagtaataaattaaggagacgagttca

SEQ ID NO: 82 - DNA, 300 bp, E. coli
  promoter (1)..(300): burden sensing promoter p(xthA)
caaaccatatgcatttaaagtgcatataaagtgaatacgtttgcgatgtgggtgaataaaaagaataaaaaacgcaatgttatgcagaagtaaaatataattctggaattgtgatcattgacgaaatttactggaaattactgcgccattctgacgcagcgcgcaccaaaagcgggcattttttgcgccatcgttgacatcattaacaatcatcgatcaaatcacttaacaacaggcggtaagcaacgcgaaattctgctaccatccacgcactctttatctgaataaatggcagcgact

SEQ ID NO: 83 - DNA, 301 bp, E. coli
  promoter (1)..(301): burden sensing promoter p(uspE)
taatatctgggcctgacggtagaaaccatcagccgtctgctgggtcgcttccagaaaagcggtatgctggcagtcaaaggtaaatacatcaccatcgaaaataacgatgcgctggcccagcttgctggtcatacgcgtaacgttgcctgatttttccgcataactcactatccttctgtcatatcattaaatttttctgatttattgatctggcagaaggttcatcactgtttcattcaccagatatgggttaatcttttaattacaaactgcgttgacagttgttgtaaggagaccctgt

SEQ ID NO: 84 - DNA, 300 bp, E. coli
  promoter (1)..(300): burden sensing promoter p(gadB)
taattttataaatgcgttcaaaataataatcaagtactaatagtgatattttaaggtctgatttttacgtgataattcaggaggcacagaatgcgcataaaaataacagcataaaacaccttaccaccacccaagaatttcatattgtattgtttttcaatgaaaaaatattattcgcgtaatatctcacgataaataacattaggattttgttatttaaacacgagtcctttgcacttgcttactttatcgataaatcctacttttttaatgcgatccaatcattttaaggagtttaaa

SEQ ID NO: 85 - DNA, 300 bp, E. coli
  promoter (1)..(300): burden sensing promoter p(ahpC)
tagatcaggtgattgccctttgtttatgagggtgttgtaatccatgtcgttgttgcatttgtaagggcaacacctcagcctgcaggcaggcactgaagataccaaagggtagttcagattacacggtcacctggaaagggggccattttactttttatcgccgctggcggtgcaaagttcacaaagttgtcttacgaaggttgtaaggtaaaacttatcgatttgataatggaaacgcattagccgaatcggcaaaaattggttaccttacatctcatcgaaaacacggaggaagtatag

SEQ ID NO: 86 - DNA, 300 bp, E. coli
  promoter (1)..(300): burden sensing promoter p(katG)
gtgatcacaaattttaaacagagcacaaaatgctgcctcgaaatgagggcgggaaaataaggttatcagccttgttttctccctcattacttgaaggatatgaagctaaaacccttttttataaagcatttgtccgaattcggacataatcaaaaaagcttaattaagatcaatttgatctacatctctttaaccaacaatatgtaagatctcaactatcgcatccgtggattaattcaattataacttctctctaacgctgtgtatcgtaacggtaacactgtagaggggagcacattg

SEQ ID NO: 87 - DNA, 300 bp, E. coli
  promoter (1)..(300): burden sensing promoter p(grxA)
tagaatctgcacttctggccgagaaaatggctcaggcagcgacagggagtcgcttaccgacagcagcgccaccgccagtagcatcattccgataaattccagtatcaacacgcctttaggcaatttaccgatcgcgcgcatacgcttccctctgcaaagtgagccttcagtctaaaacttttcactgtattgtgtttaacagttatagcttttagcaattaatgcaacaggttaaacctactttcagcgaatacattttagcgtgatcattacaggcataaatctatgaggagagaaata

SEQ ID NO: 88 - DNA, 299 bp, E. coli
  promoter (1)..(299): burden sensing promoter p(oxyS)
taactgatccaccagcagcattcccgcctgggtgaacaacactttacggctggtccgctccagcaacatcacgcccagctcatcttccagcttacgaatttgcccgctaagcgtcggctggctaacgtggcaggaatctgccgcacgccgaaaatggcggtgttcagccaatgccaccaggtactcaagatcacgaatattcattatccatcctccatcgccacgatagttcatggcgataggtagaatagcaatgaacgattatccctatcaagcattctgactgataattgctcaca

SEQ ID NO: 89 - DNA, 300 bp, E. coli
  promoter (1)..(300): burden sensing promoter p(poxB)
taggttgtcgctgcctgccgtgcgggtgtttgcggctgctgtaagacaaaagtggtttccggtgaatatacggtgagcagcacaatgacgctgaccgacgccgaaatcgctgaaggttacgtactggcctgctcctgccatccgcagggggatttggttctcgcataatcgccttatgcccgatgatattcctttcatcgggctatttaaccgttagtgcctcctttctctcccatcccttccccctccgtcagatgaactaaacttgttaccgttatcacattcaggagatggagaacc

SEQ ID NO: 90 - DNA, 299 bp, E. coli
  promoter (1)..(299): burden sensing promoter p(trxC)
tagcgggttgtgggtacgtttatcagaatcatcatcactgcggacatacatcactttgaccttgccgcttttacctttcatttcatcgttcatgcttttctccaccagcgctgcgcgaagcgcgcagattacccgaagtccgcgcggttcgccatgatttcgtaccaaagcctgcgactatcatacctattgaataaaacagattgttgtctggaacaatgtccccgataatatgtaacatattagaaacataccggcgtcgttgccgataagtctccttactcatcccgaggttagtt

SEQ ID NO: 91 - DNA, 1000 bp, S. cerevisiae
  promoter (1)..(1000): burden sensing promoter pKAR2
gtgggagtcaatcaaatcccaatcgacgctattactggacaagtcaactttattcgcaaaacaagtcctgtaatcatcaccaaaagtctcaatgaatgcttcttcattaagatactttgaccattccataggcggaaacgtgtttttatccaacactctgtcactcttggaccgtggctttggcgccctttcattttgtcttacataaaagtatctcagcagcattattgcttctttcctcaagatccccggtatactctcgtaccctgccgcactattgttcttgggcactaatgtacacgtatcatgatttactgacaagacagtaccgttgcctccaaatctctcgttgccacaaccgaacaccacctttccaatgtctaattgcttgagagcagatgcacacattatacacggttctacagtaacatatagagtaatgtctttgaacacgtcaacaactcctcgggagcccaacatcgccttgatctgatcgatccccatgaactcagcatgtgctactccagttaatgacttgttcgtatcgttcatgccataagccatcacctggccagttggcgtatgtacaaagatgcaagctaccggtgtctcatcgtggtcaagagcgtatctagccaaacggacagctgtcctcatatgtttaatatgctgcatagtgtgagtcctctagtttttaccgcagccaccagccgcttctcgagcaaagtgtagatcccattaggactcatcattcatctaattttgctatgttagctgcaactttctattttaatagaaccttctggaaatttcacccggcgcggcacccgaggaactggacagcgtgtcgaaaaagttgcttttttatataaaggacacgaaaagggttctctggaagatataaatatggctatgtaattctaaagattaacgtgttactgttttacttttttaaagtccccaagagtagtctcaagggaaaaagcgtatcaaacatacc

SEQ ID NO: 92 - DNA, 1000 bp, S. cerevisiea
  promoter (1)..(1000): burden sensing promoter pPDI1
caggtcgtcagatgtgacgttctcatcgtctagcaaatcatcgggaatcttggacttcatttgctccatggagaaagtatgatctccatgcaagttaacagaacatatacggaaattggtaccacccaggtcggcggctagtaaaacaccgcgctccgtcccgttgggtgacccggtgacgaacgccggaatcataggaagacctttgtccgaggccaatgtgtggccttcctttggtggagctagacctttttccatttgttcgatgaagtaagcagttaattcgtccagcttctcgggggtaacctcgaaatcgtcgcagatctggtccacggcctggatgaccgctctctcagtggctttgtgtaagtcgtcgaatgacatcttgtgtatgatagagttgtattagtggtggtgttgtggtttacggaagctgagttgggcactgatgggggggttgggggttctgttgatagcggatatttatatgggcgcgttttcattagtgcccaccgtttgagcgtggtgtgacaccacgcccaagatagggggccccctgaaaggggttgaccgtccgtcggcacaccacttataatgcggggtgcaagcgccgcgtctaaaattttttttttttccatttttgtcgttattgttatttcccgttttttgttttttttgattttttcggagcgacaaacctttcgaaacacgtgtcctgaaaattatcctgggctgcacgtgataatatgttaccctgtcgggcggcgcctctttttcccttttctctcactagtctctttttccaatttgccaccgtgtagcattttgttgtgctgttacaaccacaacaaaacgaaaaacccgtatggacatacatatatatatatatatatatatatattttgttacgcgtgcattttcttgttgcaagcagcatgtctaattggtaattttaaagctgccaagctctacataaagaaaaacatacatctatcccgtt

SEQ ID NO: 93 - DNA, 1000 bp, S. cerevisiae
  promoter (1)..(1000): burden sensing promoter pSSA1
cactcatatcgggggtcttacttcccatcataaacacggaccaaagaattaaattcatcattcacataagcgaaaaaaagtaatcattattagttaacttccctttacatgtaaccataggaaaaaaaaaaaagaaagaaaaacaacgatctataaagtaaactaaatcggaacatacccttcaatgtatgacttgtcagccaaagaagcgtttaattgtttcaaagtttcaatcttggagaaatcggtggatgccattatgtgtgtatatattcggttggactcttcagtgctgaaaggtagaaagcatgaggtaaaaagataaagagtagaaggaaaaaaaaaagaaccaactaaatatagtgggtagataaccttaaactatttatttagaggcgacaatgtgaaaaattttttcttcaaaggctcggttgtcgacaaattgttacgttgtgctttgatttctaaagcgcttcttcacctgcaggttctgagccctaagaaaaaaaatttccttggttgaaaatggcggaaaaaaaaaattcagaaaaagaaataaagcacgtgtgcgcggtgtgtggatgatggtttcatcattgtcaacggcattttcgttcttgtggattgttgtaaactttccagaacattctagaaagaaagcacacggaacgtttagaagctgtcatttgcgttttttctccagattttagttgagaaagtaattaaattattcttctttttccagaacgttccatcggcggcaaaagggagagaaagaacccaaaaagaaggggggccatttagattagctgatcgtttcgaggacttcaaggttatataaggggtggattgatgtatcttcgagaagggattgagttgtagtttcgtttcccaattcttacttaagttgttttattttctctatttgtaagataagcacatcaaaagaaaagtaatcaagtattacaagaaacaaaaattcaagtaaataacagataat

SEQ ID NO: 94 - DNA, 1000 bp, S. cerevisiea
  promoter (1)..(1000): burden sensing promoter pFPR2
ctgatcttttcacgcagttaggtaaggaaaatcgtggccaaataaatttcattgcattaaactctacaatgttcccacaccacgttagattcctaaatatgagagaacagttcccattatttgctatccataatatgatcaataatctgaaatatggtttaccacaactaccagaagaagagtacgcgaaattagaaaaaccacaaccactagacagagatatgatcgttcagttggtaaaagattaccgtgaaggtactgccaagccaattgttaagtcagaagagattccaaaagaacaaaagtccaatgtttataaaatagttgggaagacacatgacgacattgttcatgatgatgacaaggatgtccttgtcaaatattacgcgacatggtgtattcatagtaaaaggtttgcgcctatttacgaagaaattgcaaatgtcttagcatctgatgaatctgttcgcgataaaatcttgatcgccgaagtagattcaggggcaaatgatatcttaagttttcctgtgacaggatatccaaccattgctttgtatcctgccggaaataactctaagcctattatcttcaataaaattagaaatttggaagatgttttcgaatttatcaaggaatcaggtacacatcacattgacggccaggcaatttatgataaattgcaccaggccaaggattctgaagtgtctactgaagataccgtacatgatgaattataatcaataaataaagcatatataatgcacatttttaacatctgattactcgcatcgtttctggaagaaaatagctaatattcgttatttatggcatcacgattattctcaccagttacccgtttatgctcttgaagagatttagcattactgccagcgcatcttcaaatacaggtttatatgagacccattactataaccctaagaagagaaaaaggagtgctttcgttttcaatcacattctagtttacagtaattgagtctcg

SEQ ID NO: 95 - DNA, 1000 bp, S. cerevisiae
  promoter (1)..(1000): burden sensing promoter pRPL3
cctttcctgcgggatagcttttgcttcaggttcttctgaggttctgaaaatcaatatatttttccgacaatttctcactatgcctctatcccccttaaaaagaaacactttctaccctcttttctaaactctgcacactagaccgagacagcaaatcggagcccgagagaaaatccggaggacggaaaaactagaagtaatcttatgcggggagcatgcaccagaacgcccagaaaacgtgaatgacactacatactttgatacggatgttggtatttttccggctttttctattttatcgatgccgtgtctgctgccattacgtacaggtaggcaaaggcaaacaagaatagcactttttcacttgctgcttttttttgtgaatgaagtttatcgtatattctgttagtgccgctcgtatcagccacttacgttatcattctaaagtaagtatacgaaatgtgcaaaccttagtagacgttcaagaattgctcgataattgcgaacaaaccagctgctaagccgggaagttaagtcctcaacacagaaatgatgcaaacaatttattaaattcagtggtaatgcaacagcaagaggaaaggtggagggattaacgcatttcagacagctttatagggggaaagaaagcactcgcaaacttgctgcctgttcgcagtcattggttgcaaaaactaaactctactcacgcacactggaatgaatggcaatattcttttttaggttaaccggccggacagtaatatagtaatcgttttgtacgtttttcaagaagcgacgcacaactgttttccattttttttttttttttttcagtgatcatcgtccatgaaaaaaatttttcatttgtctctttcgtgcttcctggatatataaaatacgatttatttagttgtctttgtcaatcctcatctttctttactcattatttcatttcggttttgtcatctctagaacaacacagttactacaacaatcaatc

SEQ ID NO: 96 - DNA, 1000 bp, S. cerevisiae
  promoter (1)..(1000): burden sensing promoter pRPL6A
attctcgtgcaagcagttttgcgcgtactttagctcctcatggcacttacaatggttttattaccgtggttgctgcggaaaacgttgccaagcatgttcaaattaagatctctttaactcaaggtggtagactaaaacacatatacaaaacgaaaagccaaaaagccaataatgatggtgttgccgtatttgatgaagagtgctcgttcaaggcttctcccgaagccaatttggtactgggtgcaatttcccatcaaagactatcgagggacaaagatcttggtattgctcaaatcaacttgggtgaccctcaaattcaacaagatggccaaatttctgtaaaattaggagacggtcatctgattgtaaagattaattacggtaaagacaagaatggtcaggtacctcccgtgccagaagttcctcaagaatacacgcagtaataaacagtgaaaactattcttttatacgctcaataagggcacatttggtgtgttaacaggtgtcttttctgtgtttgttataattttgcgctattattatataacgttatatttactataatatattacaacatatattacaacatatttcaacgctctcctgttactgcttagggagaagaaagaaatgtgaagactgctattaaatccgtacattattaaaatgtatggatttgttatatttttcttcagttttttccttaaccagattcgaaaagcggcccgcctagaccattgcggttgcggctaaagcgttctggagagggcttctccgctgggcggacaacagaagcgagagacacgtttcccgtctgggaggactcaccggatttgtccagtttcccactggagtgtgctttgttccttttgcaaaatttcgttggtatggaggttatcgaatggaagggttacatgaatagattaaatgtactactcattaaagattgaatatcagttttacattaggcgaaacaacaaagtaatagccatccaacgaa

SEQ ID NO: 97 - DNA, 1000 bp, S. cerevisiae
  promoter (1)..(1000): pRPL28
  promoter (1)..(1000): burden sensing promoter pRPL28
gggatagccctccatgggaatgtcaaattctgagcacgaaagcacctgctgaggtgcatttaattccgacaagtggtaaccaaattgtattgaaccgattgaggctactataattgcataacataacgcctttgtaattttatgcttgttttgccttggcatgctaacattggatagcaacgatgcactagatagaatcctattcatactatgctacgtacctgtttaactcttctcattttatccgttttctttcttcaccgttcctcttaagttctttatttttttcataacagaatgatcacccctttcactttgccgccaatataatattaacacacaagaaataagtatgaggtagtttgctctcgaaaaaaccaagtaatagttcaaaaaatgaaaaaaagaaaacaaataccaaattatgccaccgttaccttacgtttcatggttaatcatcgtttactgccgcctatgagcgtaagctaatgttataaagaaacaagctataatattgttaaatatagttgatcaacagcattgtaatgattacaagagacgaggtggaatgaaccttatgaaatgcgtattatatataaactgtaataagagctaagttgaattgaaatctacgatacttgatgttgacattatagcactagttcccaggaaaccctttcgaaaaacacagcaaaaacaagagtactgtaaccaatgtaacatctgtacaccagggacccacacattaccaaaatcaaaattatttttctaatgcctgttatttttcctatttttcctctggcgcgtgaatagcccgcagagacgcaaacaattttcctcgcagtttttcgcttgtttaatgcgtattttcccagataggttcaaacctttcatctgtatcccgtatatttaagatggcgtttgctttctccgttgatttttttccttcttagtgatttttttgcattaaatcccagaacaatcatccaactaatcaaga

SEQ ID NO: 98 - DNA, 580 bp, S. cerevisiae
  promoter (1)..(580): burden sensing promoter pOGG1
tgcaatcaggttcttcccaatcatccgaatcagagagcaaatctaggtcttcttttgaaagtatggaaggatgcttcaattgtgcttgaataaagttattagacctgaaaccacgactactcatagaaaacgatagtttggcgtgcgatacgtttttgagtaaaagaaaactgttgaaactacagataaatggccttcttggtataatatgattcaatgttgatcttatccactttggcatgtaaaattgattgatacaagtaagctaatcgctcaatggataatattacaaataaaaatatcgaggcaataccagtatttcaatgtctggccaaataaatagtttagtacagcaatttgattaacgttaaagttactctcctctttgaataatgtcgtggttaaaaagtaaagtatttgtttatacattaagtgaagaaaattaagacgcgcctttctttaatgtaacgccaaaaattttcaagagatgagctgaacagcatcacaaaactactatttccagcggaagaaggcatttgaagcgtcctgattcataattgcgattttatttatcaaccag

SEQ ID NO: 99 - DNA, 1000 bp, S. cerevisiae
  promoter (1)..(1000): burden sensing promoter pRAD51
ccgcaataaagggcttcccggacttggaattaatacctgctaccaccggccccacaaagtatggaccgaatcttctttcataaagtgaacttgacactaattgggtaaacgtttcaggctcaatggccctttcttccttcaacttatataggttcgtcttgtagcggaacatctcgttcagagtagtcacgtcggtagccagaccggtaatccctaagaacacatgcccatagtggaagattttttcaaacttgttcgacacacctagtgactggcttccgagacgcaaatcacaggcaatggccacacagtctttacctgtcatcgcaacgacgataccaccgttaatagaacttggatccgacattttttttttatgctttattcactgttcaatattttcaccacaattcgcaagaaacgcactctacttcgaaactacggttcaaacttacttagcagcttcccgatttaattggcctttctactatgccataaactctttcttcctctcttttcatcgcccctgcatttgcacttttttgccaccggcagtgccatccggtcacatgactacaccacgttaatagcgatctggcttatcattgtcacagagtaaattaaaatggacggtaaatgttggaaatgcaccactaccgttcttcaaccaatctagtttagctatcctgcaacaggtggccttcttgagcattccctgagcattccaaccggttgtatcagtgttttatcaccgtctcaccatatcccacgactaggccacacttcgttaccctatgctacgcgtcatttccgctatttctgtcctggtttgtttacagtacgcgtggtgggaccataaaggggaatagtggggactggagaaaaaattttctcagttacttcttctatcttccgtagtttccatatactagtagttgagtgtagcgacaaagagcagacgtagttatttgttaaaggcctactaatttgttatcgtcat

SEQ ID NO: 100 - DNA, 1000 bp, S. cerevisiae
  promoter (1)..(1000): burden sensing promoter pRAD54
tgcgctacggttcctgccgctcgtgggaaccccacgcaaaacatattattcgcttctctctgctgacaactccggtttacgttataccgtattaggatcactataagggttccttcgggaggaggggggaggggaagaatgtacatcgtcataaggcctttatggtgtgaagtgggttttgcgtggaaaattcgttttcaatgatatagagcccacgcatatacgtacatactagtggccaaaagcgtggggtgggcggacaaagctacactggtaaaatacaggattctatgaacaataacaacaaccagctcacgttgctgaacagccgaggtcagccgatgcaaccgaggtttccaaagtagcatttctgtgctagctatgtctgtaggtttacatttaatggtgcgtggttccagcttcatgtgcttgcatgtgatgtcctgcagatggtaagaagattctgaaagccgcgctaggagaaaaatattctgctcgaagatctgtcctcttaagtagaaagcgtgaaattgttgcgttcttgcattactactcaacgcgtacgcaaatgcgtctactgcacctgcatgataaagcttatgtatcaaaaatttaacatcttgaaaatacacaagtggtgcaaagatgtgtcacgttctggacctgagtggtgccatgtatgctatttaacatgcaaaggggaagacccttccgccttactgcaataataaaaagtattttacgcgttacccaatatagcaaagtttcgcgcaaaaaaaaaaataaaaaacaattacaaacaaaaagaaaaaaaaggaaataatagaagatctaactgaagcgaaggccaaaactcttctcacttgacgtaatagccgatacaaaatctagagcagcaacttttctctttcttcactaaagctgctacgaaagtatagaaaaatcaaacgctcagaacttagctctatttcaaggtaccatatatatttccttataactg

SEQ ID NO: 101 - DNA, 5776 bp, synthetic
  plasmid (1)..(5776): pEG34
  CDS (463)..(1758): hGH-glycine linker-GFP
atcgatgcatgcgcccaatacgcaaaccgcctctccccgcgcgttggccgattcattaatgcagctggcacgacaggtttcccgactggaaagcgggcagtgagcgcaacgcaattaatgtgagttagctcactcattaggcaccccaggctttacactttatgcttccggctcgtatgttgtgtggaattgtgagcggataacaatttcacacaggaaacagctatgaccatgattacgccaagcgcgcaattaaccctcactaaagggaacaaaagctgggtaccgggccccccctcgaggtcgacggtatcgataagcttgatatcagctgaattcattaaagaggagaaaggtaccatgggtctgggcaagaaaaagaaactgctgctgctgttactgagcagcgcagttgcagcaagctttatgagcctgaccattagcctgcctggtgttcaggcatttccgaccattccgctgagccgtctgtttgataatgcaatgctgcgtgcacatcgtctgcatcagctggcatttgatacctatcaagaatttgaagaagcgtatatcccgaaagagcagaaatatagcttcctgcagaatccgcagaccagcctgtgttttagcgaaagcattccgacaccgagcaatcgtgaagaaacccagcagaaaagcaatctggaactgctgcgtattagtctgctgctgattcagagctggctggaaccggtgcagtttctgcgtagcgtttttgcaaatagcctggtttatggtgcaagcgatagcaatgtttatgatctgctgaaagatctggaagaaggtattcagaccctgatgggtcgtctggaagatggttcaccgcgtaccggtcagatctttaaacagacctatagcaaattcgataccaacagccataatgatgatgccctgctgaaaaactatggtctgctgtattgtttccgcaaagatatggataaagtggaaacctttctgcgcattgttcagtgtcgtagcgttgaaggtagctgtggttttggtggcatgcgtaaaggcgaagagctgttcactggtttcgtcactattctggtggaactggatggtgatgtcaacggtcataagttttccgtgcgtggcgagggtgaaggtgacgcaactaatggtaaactgacgctgaagttcatctgtactactggtaaactgccggtaccttggccgactctggtaacgacgctgacttatggtgttcagtgctttgctcgttatccggaccacatgaagcagcatgacttcttcaagtccgccatgccggaaggctatgtgcaggaacgcacgatttcctttaaggatgacggcacgtacaaaacgcgtgcggaagtgaaatttgaaggcgataccctggtaaaccgcattgagctgaaaggcattgactttaaagaagacggcaatatcctgggccataagctggaatacaattttaacagccacaatgtttacatcaccgccgataaacaaaaaaatggcattaaagcgaattttaaaattcgccacaacgtggaggatggcagcgtgcagctggctgatcactaccagcaaaacactccaatcggtgatggtcctgttctgctgccagacaatcactatctgagcacgcaaagcgttctgtctaaagatccgaacgagaaacgcgatcacatggttctgctggagttcgtaaccgcagcgggcatcacgcatggtatggatgaactgtacaaataagtcgacctgcaggcatgcaagcttggctgttttggcggatgagagaagattttcagcctgatacagattaaatcagaacgcagaagcggtctgataaaacagaatttgcctggcggcagtagcgcggtggtcccacctgaccccatgccgaactcagaagtgaaacgccgtagcgccgatggtagtgtggggtctccccatgcgagagtagggaactgccaggcatcaaataaaacgaaaggctcagtcgaaagactgggcctttcgttttatctgttgtttgtcggtgaacgctctcctgagtaggacaaatccgccgggagcggatttgaacgttgcgaagcaacggcccggagggtggcgggcaggacgcccgccataaactgccaggcatcaaattaagcagaaggccatcctgacggatggcctttttgcgtttctacaaactcttttgtttatttttctaaatacattcaaatatgtatccgctcatgagacaataaccctgataaatgcttcaataatattgaaaaaggaagagtatgagtattcaacatttccgtgtcgcccttattcccttttttgcggcattttgccttcctgtttttgctcacccagaaacgctggtgaaagtaaaagatgctgaagatcagttgggtgcagcaaactattaactggcgaactacttactctagcttcccggcaacaattaatagactggatggaggcggataaagttgcaggaccacttctgcgctcggcccttccggctggctggtttattgctgataaatctggagccggtgagcgtgggtctcgcggtatcattgcagcactggggccagatggtaagccctcccgtatcgtagttatctacacgacggggagtcaggcaactatggatgaacgaaatagacagatcgctgagataggtgcctcactgattaagcattggtaactgtcagaccaagtttactcatatatactttagattgatttacgcgccctgtagcggcgcattaagcgcggcgggtgtggtggttacgcgcagcgtgaccgctacacttgccagcgccctagcgcccgctcctttcgctttcttcccttcctttctcgccacgttcgccggctttccccgtcaagctctaaatcgggggctccctttagggttccgatttagtgctttacggcacctcgaccccaaaaaacttgatttgggtgatggttcacgtagtgggccatcgccctgatagacggtttttcgccctttgacgttggagtccacgttctttaatagtggactcttgttccaaacttgaacaacactcaaccctatctcgggctattcttttgatttataagggattttgccgatttcggcctattggttaaaaaatgagctgatttaacaaaaatttaacgcgaattttaacaaaatattaacgtttacaatttaaaaggatctaggtgaagatcctttttgataatctcatgaccaaaatcccttaacgtgagttttcgttccactgagcgtcagaccccgtagaaaagatcaaaggatcttcttgagatcctttttttctgcgcgtaatctgctgcttgcaaacaaaaaaaccaccgctaccagcggtggtttgtttgccggatcaagagctaccaactctttttccgaaggtaactggcttcagcagagcgcagataccaaatactgtccttctagtgtagccgtagttaggccaccacttcaagaactctgtagcaccgcctacatacctcgctctgctaatcctgttaccagtggggcatttgagaagcacacggtcacactgcttccggtagtcaataaaccggtaaaccagcaatagacataagcggctatttaacgaccctgccctgaaccgacgaccgggtcgaatttgctttcgaatttctgccattcatccgcttattatcacttattcaggcgtagcaccaggcgtttaagggcaccaataactgccttaaaaaaattacgccccgccctgccactcatcgcagtactgttgtaattcattaagcattctgccgacatggaagccatcacagacggcatgatgaacctgaatcgccagcggcatcagcaccttgtcgccttgcgtataatatttgcccatggtgaaaacgggggcgaagaagttgtccatattggccacgtttaaatcaaaactggtgaaactcacccagggattggctgagacgaaaaacatattctcaataaaccctttagggaaataggccaggttttcaccgtaacacgccacatcttgcgaatatatgtgtagaaactgccggaaatcgtcgtggtattcactccagagcgatgaaaacgtttcagtttgctcatggaaaacggtgtaacaagggtgaacactatcccatatcaccagctcaccgtctttcattgccatacggaattccggatgagcattcatcaggcgggcaagaatgtgaataaaggccggataaaacttgtgcttatttttctttacggtctttaaaaaggccgtaatatccagctgaacggtctggttataggtacattgagcaactgactgaaatgcctcaaaatgttctttacgatgccattgggatatatcaacggtggtatatccagtgatttttttctccattttagcttccttagctcctgaaaatctcgataactcaaaaaatacgcccggtagtgatcttatttcattatggtgaaagttggaacctcttacgtgccgatcaacgtctcattttcgccaaaagttggcccagggcttcccggtatcaacagggacaccaggatttatttattctgcgaagtgatcttccgtcacaggtatttattcggcgcaaagtgcgtcgggtgatgctgccaacttactgatttagtgtatgatggtgtttttgaggtgctccagtggcttctgtttctatcagctgtccctcctgttcagctactgacggggtggtgcgtaacggcaaaagcaccgccggacatcagcgctagcggagtgtatactggcttactatgttggcactgatgagggtgtcagtgaagtgcttcatgtggcaggagaaaaaaggctgcaccggtgcgtcagcagaatatgtgatacaggatatattccgcttcctcgctcactgactcgctacgctcggtcgttcgactgcggcgagcggaaatggcttacgaacggggcggagatttcctggaagatgccaggaagatacttaacagggaagtgagagggccgcggcaaagccgtttttccataggctccgcccccctgacaagcatcacgaaatctgacgctcaaatcagtggtggcgaaacccgacaggactataaagataccaggcgtttccccctggcggctccctcgtgcgctctcctgttcctgcctttcggtttaccggtgtcattccgctgttatggccgcgtttgtctcattccacgcctgacactcagttccgggtaggcagttcgctccaagctggactgtatgcacgaaccccccgttcagtccgaccgctgcgccttatccggtaactatcgtcttgagtccaacccggaaagacatgcaaaagcaccactggcagcagccactggtaattgatttagaggagttagtcttgaagtcatgcgccggttaaggctaaactgaaaggacaagttttggtgactgcgctcctccaagccagttacctcggttcaaagagttggtagctcagagaaccttcgaaaaaccgccctgcaaggcggttttttcgttttcagagcaagagattacgcgcagaccaaaacgatctcaagaagatcatcttattaatcagataaaatatttgctcatgagcccgaagtggcgagcccgatcttccccatcggtgatgtcggcgatataggcgccagcaaccgcacctgtggcgccggtgatgccggccacgatgcgtccggcgtagaggatctgctcatgtttgacagcttatc

SEQ ID NO: 102 - protein, 431 aa, synthetic
FPTIPLSRLFDNAMLRAHRLHQLAFDTYQEFEEAYIPKEQKYSFLQNPQTSLCFSESIPTPSNREETQQKSNLELLRISLLLIQSWLEPVQFLRSVFANSLVYGASDSNVYDLLKDLEEGIQTLMGRLEDGSPRTGQIFKQTYSKFDTNSHNDDALLKNYGLLYCFRKDMDKVETFLRIVQCRSVEGSCGFGGMRKGEELFTGFVTILVELDGDVNGHKFSVRGEGEGDATNGKLTLKFICTTGKLPVPWPTLVTTLTYGVQCFARYPDHMKQHDFFKSAMPEGYVQERTISFKDDGTYKTRAEVKFEGDTLVNRIELKGIDFKEDGNILGHKLEYNFNSHNVYITADKQKNGIKANFKIRHNVEDGSVQLADHYQQNTPIGDGPVLLPDNHYLSTQSVLSKDPNEKRDHMVLLEFVTAAGITHGMDELYK

SEQ ID NO: 103 - DNA, 660 bp, synthetic
  CDS (1)..(660): Chloramphenicol_acetyltransferase
atggagaaaaaaatcactggatataccaccgttgatatatcccaatggcatcgtaaagaacattttgaggcatttcagtcagttgctcaatgtacctataaccagaccgttcagctggatattacggcctttttaaagaccgtaaagaaaaataagcacaagttttatccggcctttattcacattcttgcccgcctgatgaatgctcatccggaattccgtatggcaatgaaagacggtgagctggtgatatgggatagtgttcacccttgttacaccgttttccatgagcaaactgaaacgttttcatcgctctggagtgaataccacgacgatttccggcagtttctacacatatattcgcaagatgtggcgtgttacggtgaaaacctggcctatttccctaaagggtttattgagaatatgtttttcgtctcagccaatccctgggtgagtttcaccagttttgatttaaacgtggccaatatggacaacttcttcgcccccgttttcaccatgggcaaatattatacgcaaggcgacaaggtgctgatgccgctggcgattcaggttcatcatgccgtctgtgatggcttccatgtcggcagaatgcttaatgaattacaacagtactgcgatgagtggcagggcggggcgtaa

SEQ ID NO: 104 - protein, 219 aa, synthetic
MEKKITGYTTVDISQWHRKEHFEAFQSVAQCTYNQTVQLDITAFLKTVKKNKHKFYPAFIHILARLMNAHPEFRMAMKDGELVIWDSVHPCYTVFHEQTETFSSLWSEYHDDFRQFLHIYSQDVACYGENLAYFPKGFIENMFFVSANPWVSFTSFDLNVANMDNFFAPVFTMGKYYTQGDKVLMPLAIQVHHAVCDGFHVGRMLNELQQYCDEWQGGA

SEQ ID NO: 105 - DNA, 4347 bp, synthetic
  plasmid (1)..(4347): pEG0
atcgatgcatgcgcccaatacgcaaaccgcctctccccgcgcgttggccgattcattaatgcagctggcacgacaggtttcccgactggaaagcgggcagtgagcgcaacgcaattaatgtgagttagctcactcattaggcaccccaggctttacactttatgcttccggctcgtatgttgtgtggaattgtgagcggataacaatttcacacaggaaacagctatgaccatgattacgccaagcgcgcaattaaccctcactaaagggaacaaaagctgggtaccgggccccccctcgaggtcgacggtatcgataagcttgatatcgaattcctgcaggcatgcaagcttggctgttttggcggatgagagaagattttcagcctgatacagattaaatcagaacgcagaagcggtctgataaaacagaatttgcctggcggcagtagcgcggtggtcccacctgaccccatgccgaactcagaagtgaaacgccgtagcgccgatggtagtgtggggtctccccatgcgagagtagggaactgccaggcatcaaataaaacgaaaggctcagtcgaaagactgggcctttcgttttatctgttgtttgtcggtgaacgctctcctgagtaggacaaatccgccgggagcggatttgaacgttgcgaagcaacggcccggagggtggcgggcaggacgcccgccataaactgccaggcatcaaattaagcagaaggccatcctgacggatggcctttttgcgtttctacaaactcttttgtttatttttctaaatacattcaaatatgtatccgctcatgagacaataaccctgataaatgcttcaataatattgaaaaaggaagagtatgagtattcaacatttccgtgtcgcccttattcccttttttgcggcattttgccttcctgtttttgctcacccagaaacgctggtgaaagtaaaagatgctgaagatcagttgggtgcagcaaactattaactggcgaactacttactctagcttcccggcaacaattaatagactggatggaggcggataaagttgcaggaccacttctgcgctcggcccttccggctggctggtttattgctgataaatctggagccggtgagcgtgggtctcgcggtatcattgcagcactggggccagatggtaagccctcccgtatcgtagttatctacacgacggggagtcaggcaactatggatgaacgaaatagacagatcgctgagataggtgcctcactgattaagcattggtaactgtcagaccaagtttactcatatatactttagattgatttacgcgccctgtagcggcgcattaagcgcggcgggtgtggtggttacgcgcagcgtgaccgctacacttgccagcgccctagcgcccgctcctttcgctttcttcccttcctttctcgccacgttcgccggctttccccgtcaagctctaaatcgggggctccctttagggttccgatttagtgctttacggcacctcgaccccaaaaaacttgatttgggtgatggttcacgtagtgggccatcgccctgatagacggtttttcgccctttgacgttggagtccacgttctttaatagtggactcttgttccaaacttgaacaacactcaaccctatctcgggctattcttttgatttataagggattttgccgatttcggcctattggttaaaaaatgagctgatttaacaaaaatttaacgcgaattttaacaaaatattaacgtttacaatttaaaaggatctaggtgaagatcctttttgataatctcatgaccaaaatcccttaacgtgagttttcgttccactgagcgtcagaccccgtagaaaagatcaaaggatcttcttgagatcctttttttctgcgcgtaatctgctgcttgcaaacaaaaaaaccaccgctaccagcggtggtttgtttgccggatcaagagctaccaactctttttccgaaggtaactggcttcagcagagcgcagataccaaatactgtccttctagtgtagccgtagttaggccaccacttcaagaactctgtagcaccgcctacatacctcgctctgctaatcctgttaccagtggggcatttgagaagcacacggtcacactgcttccggtagtcaataaaccggtaaaccagcaatagacataagcggctatttaacgaccctgccctgaaccgacgaccgggtcgaatttgctttcgaatttctgccattcatccgcttattatcacttattcaggcgtagcaccaggcgtttaagggcaccaataactgccttaaaaaaattacgccccgccctgccactcatcgcagtactgttgtaattcattaagcattctgccgacatggaagccatcacagacggcatgatgaacctgaatcgccagcggcatcagcaccttgtcgccttgcgtataatatttgcccatggtgaaaacgggggcgaagaagttgtccatattggccacgtttaaatcaaaactggtgaaactcacccagggattggctgagacgaaaaacatattctcaataaaccctttagggaaataggccaggttttcaccgtaacacgccacatcttgcgaatatatgtgtagaaactgccggaaatcgtcgtggtattcactccagagcgatgaaaacgtttcagtttgctcatggaaaacggtgtaacaagggtgaacactatcccatatcaccagctcaccgtctttcattgccatacggaattccggatgagcattcatcaggcgggcaagaatgtgaataaaggccggataaaacttgtgcttatttttctttacggtctttaaaaaggccgtaatatccagctgaacggtctggttataggtacattgagcaactgactgaaatgcctcaaaatgttctttacgatgccattgggatatatcaacggtggtatatccagtgatttttttctccattttagcttccttagctcctgaaaatctcgataactcaaaaaatacgcccggtagtgatcttatttcattatggtgaaagttggaacctcttacgtgccgatcaacgtctcattttcgccaaaagttggcccagggcttcccggtatcaacagggacaccaggatttatttattctgcgaagtgatcttccgtcacaggtatttattcggcgcaaagtgcgtcgggtgatgctgccaacttactgatttagtgtatgatggtgtttttgaggtgctccagtggcttctgtttctatcagctgtccctcctgttcagctactgacggggtggtgcgtaacggcaaaagcaccgccggacatcagcgctagcggagtgtatactggcttactatgttggcactgatgagggtgtcagtgaagtgcttcatgtggcaggagaaaaaaggctgcaccggtgcgtcagcagaatatgtgatacaggatatattccgcttcctcgctcactgactcgctacgctcggtcgttcgactgcggcgagcggaaatggcttacgaacggggcggagatttcctggaagatgccaggaagatacttaacagggaagtgagagggccgcggcaaagccgtttttccataggctccgcccccctgacaagcatcacgaaatctgacgctcaaatcagtggtggcgaaacccgacaggactataaagataccaggcgtttccccctggcggctccctcgtgcgctctcctgttcctgcctttcggtttaccggtgtcattccgctgttatggccgcgtttgtctcattccacgcctgacactcagttccgggtaggcagttcgctccaagctggactgtatgcacgaaccccccgttcagtccgaccgctgcgccttatccggtaactatcgtcttgagtccaacccggaaagacatgcaaaagcaccactggcagcagccactggtaattgatttagaggagttagtcttgaagtcatgcgccggttaaggctaaactgaaaggacaagttttggtgactgcgctcctccaagccagttacctcggttcaaagagttggtagctcagagaaccttcgaaaaaccgccctgcaaggcggttttttcgttttcagagcaagagattacgcgcagaccaaaacgatctcaagaagatcatcttattaatcagataaaatatttgctcatgagcccgaagtggcgagcccgatcttccccatcggtgatgtcggcgatataggcgccagcaaccgcacctgtggcgccggtgatgccggccacgatgcgtccggcgtagaggatctgctcatgtttgacagcttatc

SEQ ID NO: 106 - DNA, 6076 bp, synthetic
  plasmid (1)..(6076): pENDU5CAM
  CDS (108)..(911): ompA-lysostaphin
gatctcgatcccgcgaaattaatacgactcactataggggaattgtgagcggataacaattcccctctagaaataattttgtttaactttaagaaggagatatacatatgaaaaagacagctatcgcgattgcagtggcactggctggtttcgctaccgtagcgcaggctgcagcaacccatgaacatagcgcacagtggctgaataattacaaaaaaggttatggctatggtccgtatccgctgggtattaatggtggtatgcattatggtgtggatttctttatgaatattggcacaccggttaaagcaattagcagcggtaaaattgttgaagcaggttggagcaattatggtggtggtaatcagattggcctgattgaaaatgatggtgttcatcgtcagtggtatatgcatctgagcaaatacaatgtgaaagtgggcgattatgttaaagccggtcagattattggttggagcggtagcaccggttatagtaccgcaccgcatctgcattttcagcgtatggttaatagctttagcaatagcaccgcacaggatccgatgccgtttctgaaaagcgcaggttatggtaaagcaggcggtacagttaccccgacaccgaataccggttggaaaaccaacaaatatggcaccctgtataaaagcgaaagcgcaagctttaccccgaatacagatattatcacccgtaccaccggtccgtttcgtagcatgccgcagagcggtgttctgaaagcaggtcagaccattcattatgatgaagtgatgaaacaggatggtcatgtttgggttggttataccggtaatagcggtcagcgtatttatctgccggttcgtacctggaataaaagcaccaatacactgggtgttctgtggggcaccatcaaataatgagatccggctgctaacaaagcccgaaaggaagctgagttggctgctgccaccgctgagcaataactagcataaccccttggggcctctaaacgggtcttgaggggttttttgctgaaaggaggaactatatccggattggcgaatgggacgcgccctgtagcggcgcattaagcgcggcgggtgtggtggttacgcgcagcgtgaccgctacacttgccagcgccctagcgcccgctcctttcgctttcttcccttcctttctcgccacgttcgccggctttccccgtcaagctctaaatcgggggctccctttagggttccgatttagtgctttacggcacctcgaccccaaaaaacttgattagggtgatggttcacgtagtgggccatcgccctgatagacggtttttcgccctttgacgttggagtccacgttctttaatagtggactcttgttccaaactggaacaacactcaaccctatctcggtctattcttttgatttataagggattttgccgatttcggcctattggttaaaaaatgagctgatttaacaaaaatttaacgcgaattttaacaaaatattaacgtttacaatttcaggtggcacttttcggggaaatgtgcgcggaacccctatttgtttatttttctaaatacattcaaatatgtatccgctcaataactgccttaaaaaaattacgccccgccctgccactcatcgcagtactgttgtaattcattaagcattctgccgacatggaagccatcacagacggcatgatgaacctgaatcgccagcggcatcagcaccttgtcgccttgcgtataatatttgcccatggtgaaaacgggggcgaagaagttgtccatattggccacgtttaaatcaaaactggtgaaactcacccagggattggctgagacgaaaaacatattctcaataaaccctttagggaaataggccaggttttcaccgtaacacgccacatcttgcgaatatatgtgtagaaactgccggaaatcgtcgtggtattcactccagagcgatgaaaacgtttcagtttgctcatggaaaacggtgtaacaagggtgaacactatcccatatcaccagctcaccgtctttcattgccatacggaattccggatgagcattcatcaggcgggcaagaatgtgaataaaggccggataaaacttgtgcttatttttctttacggtctttaaaaaggccgtaatatccagctgaacggtctggttataggtacattgagcaactgactgaaatgcctcaaaatgttctttacgatgccattgggatatatcaacggtggtatatccagtgatttttttctccattttagcttccttagctcctgaaaatctcgataactcaaaaaatacgcccggtagtgatcttatttcattatggtgaaagttggaacctcttacgtgccgatcaacgtctcattttcgccaaaagttggcccagggcttcccggtatcaacagggacaccaggatttatttattctgcgaagtgatcttccgtcacaggtatttattcggcgcaaagtgcgtcattgttcatgaccaaaatcccttaacgtgagttttcgttccactgagcgtcagaccccgtagaaaagattgttcatgaccaaaatcccttaacgtgatcaaaggatcttcttgagatcctttttttctgcgcgtaatctgctgcttgcaaacaaaaaaaccaccgctaccagcggtggtttgtttgccggatcaagagctaccaactctttttccgaaggtaactggcttcagcagagcgcagataccaaatactgtccttctagtgtagccgtagttaggccaccacttcaagaactctgtagcaccgcctacatacctcgctctgctaatcctgttaccagtggctgctgccagtggcgataagtcgtgtcttaccgggttggactcaagacgatagttaccggataaggcgcagcggtcgggctgaacggggggttcgtgcacacagcccagcttggagcgaacgacctacaccgaactgagatacctacagcgtgagctatgagaaagcgccacgcttcccgaagggagaaaggcggacaggtatccggtaagcggcagggtcggaacaggagagcgcacgagggagcttccagggggaaacgcctggtatctttatagtcctgtcgggtttcgccacctctgacttgagcgtcgatttttgtgatgctcgtcaggggggcggagcctatggaaaaacgccagcaacgcggcctttttacggttcctggccttttgctggccttttgctcacatgttctttcctgcgttatcccctgattctgtggataaccgtattaccgcctttgagtgagctgataccgctcgccgcagccgaacgaccgagcgcagcgagtcagtgagcgaggaagcggaagagcgcctgatgcggtattttctccttacgcatctgtgcggtatttcacaccgcatatatggtgcactctcagtacaatctgctctgatgccgcatagttaagccagtatacactccgctatcgctacgtgactgggtcatggctgcgccccgacacccgccaacacccgctgacgcgccctgacgggcttgtctgctcccggcatccgcttacagacaagctgtgaccgtctccgggagctgcatgtgtcagaggttttcaccgtcatcaccgaaacgcgcgaggcagctgcggtaaagctcatcagcgtggtcgtgaagcgattcacagatgtctgcctgttcatccgcgtccagctcgttgagtttctccagaagcgttaatgtctggcttctgataaagcgggccatgttaagggcggttttttcctgtttggtcactgatgcctccgtgtaagggggatttctgttcatgggggtaatgataccgatgaaacgagagaggatgctcacgatacgggttactgatgatgaacatgcccggttactggaacgttgtgagggtaaacaactggcggtatggatgcggcgggaccagagaaaaatcactcagggtcaatgccagcgcttcgttaatacagatgtaggtgttccacagggtagccagcagcatcctgcgatgcagatccggaacataatggtgcagggcgctgacttccgcgtttccagactttacgaaacacggaaaccgaagaccattcatgttgttgctcaggtcgcagacgttttgcagcagcagtcgcttcacgttcgctcgcgtatcggtgattcattctgctaaccagtaaggcaaccccgccagcctagccgggtcctcaacgacaggagcacgatcatgcgcacccgtggggccgccatgccggcgataatggcctgcttctcgccgaaacgtttggtggcgggaccagtgacgaaggcttgagcgagggcgtgcaagattccgaataccgcaagcgacaggccgatcatcgtcgcgctccagcgaaagcggtcctcgccgaaaatgacccagagcgctgccggcacctgtcctacgagttgcatgataaagaagacagtcataagtgcggcgacgatagtcatgccccgcgcccaccggaaggagctgactgggttgaaggctctcaagggcatcggtcgagatcccggtgcctaatgagtgagctaacttacattaattgcgttgcgctcactgcccgctttccagtcgggaaacctgtcgtgccagctgcattaatgaatcggccaacgcgcggggagaggcggtttgcgtattgggcgccagggtggtttttcttttcaccagtgagacgggcaacagctgattgcccttcaccgcctggccctgagagagttgcagcaagcggtccacgctggtttgccccagcaggcgaaaatcctgtttgatggtggttaacggcgggatataacatgagctgtcttcggtatcgtcgtatcccactaccgagatatccgcaccaacgcgcagcccggactcggtaatggcgcgcattgcgcccagcgccatctgatcgttggcaaccagcatcgcagtgggaacgatgccctcattcagcatttgcatggtttgttgaaaaccggacatggcactccagtcgccttcccgttccgctatcggctgaatttgattgcgagtgagatatttatgccagccagccagacgcagacgcgccgagacagaacttaatgggcccgctaacagcgcgatttgctggtgacccaatgcgaccagatgctccacgcccagtcgcgtaccgtcttcatgggagaaaataatactgttgatgggtgtctggtcagagacatcaagaaataacgccggaacattagtgcaggcagcttccacagcaatggcatcctggtcatccagcggatagttaatgatcagcccactgacgcgttgcgcgagaagattgtgcaccgccgctttacaggcttcgacgccgcttcgttctaccatcgacaccaccacgctggcacccagttgatcggcgcgagatttaatcgccgcgacaatttgcgacggcgcgtgcagggccagactggaggtggcaacgccaatcagcaacgactgtttgcccgccagttgttgtgccacgcggttgggaatgtaattcagctccgccatcgccgcttccactttttcccgcgttttcgcagaaacgtggctggcctggttcaccacgcgggaaacggtctgataagagacaccggcatactctgcgacatcgtataacgttactggtttcacattcaccaccctgaattgactctcttccgggcgctatcatgccataccgcgaaaggttttgcgccattcgatggtgtccgggatctcgacgctctcccttatgcgactcctgcattaggaagcagcccagtagtaggttgaggccgttgagcaccgccgccgcaaggaatggtgcatgcaaggagatggcgcccaacagtcccccggccacggggcctgccaccatacccacgccgaaacaagcgctcatgagcccgaagtggcgagcccgatcttccccatcggtgatgtcggcgatataggcgccagcaaccgcacctgtggcgccggtgatgccggccacgatgcgtccggcgtagaggatcga

SEQ ID NO: 107 - protein, 267 aa, synthetic
MKKTAIAIAVALAGFATVAQAAATHEHSAQWLNNYKKGYGYGPYPLGINGGMHYGVDFFMNIGTPVKAISSGKIVEAGWSNYGGGNQIGLIENDGVHRQWYMHLSKYNVKVGDYVKAGQIIGWSGSTGYSTAPHLHFQRMVNSFSNSTAQDPMPFLKSAGYGKAGGTVTPTPNTGWKTNKYGTLYKSESASFTPNTDIITRTTGPFRSMPQSGVLKAGQTIHYDEVMKQDGHVWVGYTGNSGQRIYLPVRTWNKSTNTLGVLWGTIK

SEQ ID NO: 108 - DNA, 8593 bp, synthetic
  plasmid (1)..(8593): pMevT
  CDS (380)..(1564): Acetyl-CoA_acetyltransferase
  CDS (1578)..(3053): 3-hydroxy-3-methylglutaryl-coenzyme_A_synthase
  CDS (3067)..(4575): N-Terminally_Truncated_3-Hydroxy-3-Methylglutaryl_Coenzyme_A_Redu ctase
atcgatgcatgcgcccaatacgcaaaccgcctctccccgcgcgttggccgattcattaatgcagctggcacgacaggtttcccgactggaaagcgggcagtgagcgcaacgcaattaatgtgagttagctcactcattaggcaccccaggctttacactttatgcttccggctcgtatgttgtgtggaattgtgagcggataacaatttcacacaggaaacagctatgaccatgattacgccaagcgcgcaattaaccctcactaaagggaacaaaagctgggtaccgggccccccctcgaggtcgacggtatcgataagcttgatatcgaattcctgcagcccggggatcctctagagtcgactaggaggaatataaaatgaaaaattgtgtcatcgtcagtgcggtacgtactgctatcggtagttttaacggttcactcgcttccaccagcgccatcgacctgggggcgacagtaattaaagccgccattgaacgtgcaaaaatcgattcacaacacgttgatgaagtgattatgggtaacgtgttacaagccgggctggggcaaaatccggcgcgtcaggcactgttaaaaagcgggctggcagaaacggtgtgcggattcacggtcaataaagtatgtggttcgggtcttaaaagtgtggcgcttgccgcccaggccattcaggcaggtcaggcgcagagcattgtggcggggggtatggaaaatatgagtttagccccctacttactcgatgcaaaagcacgctctggttatcgtcttggagacggacaggtttatgacgtaatcctgcgcgatggcctgatgtgcgccacccatggttatcatatggggattaccgccgaaaacgtggctaaagagtacggaattacccgtgaaatgcaggatgaactggcgctacattcacagcgtaaagcggcagccgcaattgagtccggtgcttttacagccgaaatcgtcccggtaaatgttgtcactcgaaagaaaaccttcgtcttcagtcaagacgaattcccgaaagcgaattcaacggctgaagcgttaggtgcattgcgcccggccttcgataaagcaggaacagtcaccgctgggaacgcgtctggtattaacgacggtgctgccgctctggtgattatggaagaatctgcggcgctggcagcaggccttacccccctggctcgcattaaaagttatgccagcggtggcgtgccccccgcattgatgggtatggggccagtacctgccacgcaaaaagcgttacaactggcggggctgcaactggcggatattgatctcattgaggctaatgaagcatttgctgcacagttccttgccgttgggaaaaacctgggctttgattctgagaaagtgaatgtcaacggcggggccatcgcgctcgggcatcctatcggtgccagtggtgctcgtattctggtcacactattacatgccatgcaggcacgcgataaaacgctggggctggcaacactgtgcattggcggcggtcagggaattgcgatggtgattgaacggttgaattaaggaggacagctaaatgaaactctcaactaaactttgttggtgtggtattaaaggaagacttaggccgcaaaagcaacaacaattacacaatacaaacttgcaaatgactgaactaaaaaaacaaaagaccgctgaacaaaaaaccagacctcaaaatgtcggtattaaaggtatccaaatttacatcccaactcaatgtgtcaaccaatctgagctagagaaatttgatggcgtttctcaaggtaaatacacaattggtctgggccaaaccaacatgtcttttgtcaatgacagagaagatatctactcgatgtccctaactgttttgtctaagttgatcaagagttacaacatcgacaccaacaaaattggtagattagaagtcggtactgaaactctgattgacaagtccaagtctgtcaagtctgtcttgatgcaattgtttggtgaaaacactgacgtcgaaggtattgacacgcttaatgcctgttacggtggtaccaacgcgttgttcaactctttgaactggattgaatctaacgcatgggatggtagagacgccattgtagtttgcggtgatattgccatctacgataagggtgccgcaagaccaaccggtggtgccggtactgttgctatgtggatcggtcctgatgctccaattgtatttgactctgtaagagcttcttacatggaacacgcctacgatttttacaagccagatttcaccagcgaatatccttacgtcgatggtcatttttcattaacttgttacgtcaaggctcttgatcaagtttacaagagttattccaagaaggctatttctaaagggttggttagcgatcccgctggttcggatgctttgaacgttttgaaatatttcgactacaacgttttccatgttccaacctgtaaattggtcacaaaatcatacggtagattactatataacgatttcagagccaatcctcaattgttcccagaagttgacgccgaattagctactcgcgattatgacgaatctttaaccgataagaacattgaaaaaacttttgttaatgttgctaagccattccacaaagagagagttgcccaatctttgattgttccaacaaacacaggtaacatgtacaccgcatctgtttatgccgcctttgcatctctattaaactatgttggatctgacgacttacaaggcaagcgtgttggtttattttcttacggttccggtttagctgcatctctatattcttgcaaaattgttggtgacgtccaacatattatcaaggaattagatattactaacaaattagccaagagaatcaccgaaactccaaaggattacgaagctgccatcgaattgagagaaaatgcccatttgaagaagaacttcaaacctcaaggttccattgagcatttgcaaagtggtgtttactacttgaccaacatcgatgacaaatttagaagatcttacgatgttaaaaaataaggaggattacactatggttttaaccaataaaacagtcatttctggatcgaaagtcaaaagtttatcatctgcgcaatcgagctcatcaggaccttcatcatctagtgaggaagatgattcccgcgatattgaaagcttggataagaaaatacgtcctttagaagaattagaagcattattaagtagtggaaatacaaaacaattgaagaacaaagaggtcgctgccttggttattcacggtaagttacctttgtacgctttggagaaaaaattaggtgatactacgagagcggttgcggtacgtaggaaggctctttcaattttggcagaagctcctgtattagcatctgatcgtttaccatataaaaattatgactacgaccgcgtatttggcgcttgttgtgaaaatgttataggttacatgcctttgcccgttggtgttataggccccttggttatcgatggtacatcttatcatataccaatggcaactacagagggttgtttggtagcttctgccatgcgtggctgtaaggcaatcaatgctggcggtggtgcaacaactgttttaactaaggatggtatgacaagaggcccagtagtccgtttcccaactttgaaaagatctggtgcctgtaagatatggttagactcagaagagggacaaaacgcaattaaaaaagcttttaactctacatcaagatttgcacgtctgcaacatattcaaacttgtctagcaggagatttactcttcatgagatttagaacaactactggtgacgcaatgggtatgaatatgatttctaaaggtgtcgaatactcattaaagcaaatggtagaagagtatggctgggaagatatggaggttgtctccgtttctggtaactactgtaccgacaaaaaaccagctgccatcaactggatcgaaggtcgtggtaagagtgtcgtcgcagaagctactattcctggtgatgttgtcagaaaagtgttaaaaagtgatgtttccgcattggttgagttgaacattgctaagaatttggttggatctgcaatggctgggtctgttggtggatttaacgcacatgcagctaatttagtgacagctgttttcttggcattaggacaagatcctgcacaaaatgttgaaagttccaactgtataacattgatgaaagaagtggacggtgatttgagaatttccgtatccatgccatccatcgaagtaggtaccatcggtggtggtactgttctagaaccacaaggtgccatgttggacttattaggtgtaagaggcccgcatgctaccgctcctggtaccaacgcacgtcaattagcaagaatagttgcctgtgccgtcttggcaggtgaattatccttatgtgctgccctagcagccggccatttggttcaaagtcatatgacccacaacaggaaacctgctgaaccaacaaaacctaacaatttggacgccactgatataaatcgtttgaaagatgggtccgtcacctgcattaaatcctaagtcgacctgcaggcatgcaagcttggctgttttggcggatgagagaagattttcagcctgatacagattaaatcagaacgcagaagcggtctgataaaacagaatttgcctggcggcagtagcgcggtggtcccacctgaccccatgccgaactcagaagtgaaacgccgtagcgccgatggtagtgtggggtctccccatgcgagagtagggaactgccaggcatcaaataaaacgaaaggctcagtcgaaagactgggcctttcgttttatctgttgtttgtcggtgaacgctctcctgagtaggacaaatccgccgggagcggatttgaacgttgcgaagcaacggcccggagggtggcgggcaggacgcccgccataaactgccaggcatcaaattaagcagaaggccatcctgacggatggcctttttgcgtttctacaaactcttttgtttatttttctaaatacattcaaatatgtatccgctcatgagacaataaccctgataaatgcttcaataatattgaaaaaggaagagtatgagtattcaacatttccgtgtcgcccttattcccttttttgcggcattttgccttcctgtttttgctcacccagaaacgctggtgaaagtaaaagatgctgaagatcagttgggtgcagcaaactattaactggcgaactacttactctagcttcccggcaacaattaatagactggatggaggcggataaagttgcaggaccacttctgcgctcggcccttccggctggctggtttattgctgataaatctggagccggtgagcgtgggtctcgcggtatcattgcagcactggggccagatggtaagccctcccgtatcgtagttatctacacgacggggagtcaggcaactatggatgaacgaaatagacagatcgctgagataggtgcctcactgattaagcattggtaactgtcagaccaagtttactcatatatactttagattgatttacgcgccctgtagcggcgcattaagcgcggcgggtgtggtggttacgcgcagcgtgaccgctacacttgccagcgccctagcgcccgctcctttcgctttcttcccttcctttctcgccacgttcgccggctttccccgtcaagctctaaatcgggggctccctttagggttccgatttagtgctttacggcacctcgaccccaaaaaacttgatttgggtgatggttcacgtagtgggccatcgccctgatagacggtttttcgccctttgacgttggagtccacgttctttaatagtggactcttgttccaaacttgaacaacactcaaccctatctcgggctattcttttgatttataagggattttgccgatttcggcctattggttaaaaaatgagctgatttaacaaaaatttaacgcgaattttaacaaaatattaacgtttacaatttaaaaggatctaggtgaagatcctttttgataatctcatgaccaaaatcccttaacgtgagttttcgttccactgagcgtcagaccccgtagaaaagatcaaaggatcttcttgagatcctttttttctgcgcgtaatctgctgcttgcaaacaaaaaaaccaccgctaccagcggtggtttgtttgccggatcaagagctaccaactctttttccgaaggtaactggcttcagcagagcgcagataccaaatactgtccttctagtgtagccgtagttaggccaccacttcaagaactctgtagcaccgcctacatacctcgctctgctaatcctgttaccagtggggcatttgagaagcacacggtcacactgcttccggtagtcaataaaccggtaaaccagcaatagacataagcggctatttaacgaccctgccctgaaccgacgaccgggtcgaatttgctttcgaatttctgccattcatccgcttattatcacttattcaggcgtagcaccaggcgtttaagggcaccaataactgccttaaaaaaattacgccccgccctgccactcatcgcagtactgttgtaattcattaagcattctgccgacatggaagccatcacagacggcatgatgaacctgaatcgccagcggcatcagcaccttgtcgccttgcgtataatatttgcccatggtgaaaacgggggcgaagaagttgtccatattggccacgtttaaatcaaaactggtgaaactcacccagggattggctgagacgaaaaacatattctcaataaaccctttagggaaataggccaggttttcaccgtaacacgccacatcttgcgaatatatgtgtagaaactgccggaaatcgtcgtggtattcactccagagcgatgaaaacgtttcagtttgctcatggaaaacggtgtaacaagggtgaacactatcccatatcaccagctcaccgtctttcattgccatacggaattccggatgagcattcatcaggcgggcaagaatgtgaataaaggccggataaaacttgtgcttatttttctttacggtctttaaaaaggccgtaatatccagctgaacggtctggttataggtacattgagcaactgactgaaatgcctcaaaatgttctttacgatgccattgggatatatcaacggtggtatatccagtgatttttttctccattttagcttccttagctcctgaaaatctcgataactcaaaaaatacgcccggtagtgatcttatttcattatggtgaaagttggaacctcttacgtgccgatcaacgtctcattttcgccaaaagttggcccagggcttcccggtatcaacagggacaccaggatttatttattctgcgaagtgatcttccgtcacaggtatttattcggcgcaaagtgcgtcgggtgatgctgccaacttactgatttagtgtatgatggtgtttttgaggtgctccagtggcttctgtttctatcagctgtccctcctgttcagctactgacggggtggtgcgtaacggcaaaagcaccgccggacatcagcgctagcggagtgtatactggcttactatgttggcactgatgagggtgtcagtgaagtgcttcatgtggcaggagaaaaaaggctgcaccggtgcgtcagcagaatatgtgatacaggatatattccgcttcctcgctcactgactcgctacgctcggtcgttcgactgcggcgagcggaaatggcttacgaacggggcggagatttcctggaagatgccaggaagatacttaacagggaagtgagagggccgcggcaaagccgtttttccataggctccgcccccctgacaagcatcacgaaatctgacgctcaaatcagtggtggcgaaacccgacaggactataaagataccaggcgtttccccctggcggctccctcgtgcgctctcctgttcctgcctttcggtttaccggtgtcattccgctgttatggccgcgtttgtctcattccacgcctgacactcagttccgggtaggcagttcgctccaagctggactgtatgcacgaaccccccgttcagtccgaccgctgcgccttatccggtaactatcgtcttgagtccaacccggaaagacatgcaaaagcaccactggcagcagccactggtaattgatttagaggagttagtcttgaagtcatgcgccggttaaggctaaactgaaaggacaagttttggtgactgcgctcctccaagccagttacctcggttcaaagagttggtagctcagagaaccttcgaaaaaccgccctgcaaggcggttttttcgttttcagagcaagagattacgcgcagaccaaaacgatctcaagaagatcatcttattaatcagataaaatatttgctcatgagcccgaagtggcgagcccgatcttccccatcggtgatgtcggcgatataggcgccagcaaccgcacctgtggcgccggtgatgccggccacgatgcgtccggcgtagaggatctgctcatgtttgacagcttatc

SEQ ID NO: 109 - protein, 394 aa, synthetic
MKNCVIVSAVRTAIGSFNGSLASTSAIDLGATVIKAAIERAKIDSQHVDEVIMGNVLQAGLGQNPARQALLKSGLAETVCGFTVNKVCGSGLKSVALAAQAIQAGQAQSIVAGGMENMSLAPYLLDAKARSGYRLGDGQVYDVILRDGLMCATHGYHMGITAENVAKEYGITREMQDELALHSQRKAAAAIESGAFTAEIVPVNVVTRKKTFVFSQDEFPKANSTAEALGALRPAFDKAGTVTAGNASGINDGAAALVIMEESAALAAGLTPLARIKSYASGGVPPALMGMGPVPATQKALQLAGLQLADIDLIEANEAFAAQFLAVGKNLGFDSEKVNVNGGAIALGHPIGASGARILVTLLHAMQARDKTLGLATLCIGGGQGIAMVIERLN

SEQ ID NO: 110 - protein, 491 aa, synthetic
MKLSTKLCWCGIKGRLRPQKQQQLHNTNLQMTELKKQKTAEQKTRPQNVGIKGIQIYIPTQCVNQSELEKFDGVSQGKYTIGLGQTNMSFVNDREDIYSMSLTVLSKLIKSYNIDTNKIGRLEVGTETLIDKSKSVKSVLMQLFGENTDVEGIDTLNACYGGTNALFNSLNWIESNAWDGRDAIVVCGDIAIYDKGAARPTGGAGTVAMWIGPDAPIVFDSVRASYMEHAYDFYKPDFTSEYPYVDGHFSLTCYVKALDQVYKSYSKKAISKGLVSDPAGSDALNVLKYFDYNVFHVPTCKLVTKSYGRLLYNDFRANPQLFPEVDAELATRDYDESLTDKNIEKTFVNVAKPFHKERVAQSLIVPTNTGNMYTASVYAAFASLLNYVGSDDLQGKRVGLFSYGSGLAASLYSCKIVGDVQHIIKELDITNKLAKRITETPKDYEAAIELRENAHLKKNFKPQGSIEHLQSGVYYLTNIDDKFRRSYDVKK

SEQ ID NO: 111 - protein, 502 aa, synthetic
MVLTNKTVISGSKVKSLSSAQSSSSGPSSSSEEDDSRDIESLDKKIRPLEELEALLSSGNTKQLKNKEVAALVIHGKLPLYALEKKLGDTTRAVAVRRKALSILAEAPVLASDRLPYKNYDYDRVFGACCENVIGYMPLPVGVIGPLVIDGTSYHIPMATTEGCLVASAMRGCKAINAGGGATTVLTKDGMTRGPVVRFPTLKRSGACKIWLDSEEGQNAIKKAFNSTSRFARLQHIQTCLAGDLLFMRFRTTTGDAMGMNMISKGVEYSLKQMVEEYGWEDMEVVSVSGNYCTDKKPAAINWIEGRGKSVVAEATIPGDVVRKVLKSDVSALVELNIAKNLVGSAMAGSVGGFNAHAANLVTAVFLALGQDPAQNVESSNCITLMKEVDGDLRISVSMPSIEVGTIGGGTVLEPQGAMLDLLGVRGPHATAPGTNARQLARIVACAVLAGELSLCAALAAGHLVQSHMTHNRKPAEPTKPNNLDATDINRLKDGSVTCIKS

SEQ ID NO: 112 - DNA, 32 bp, synthetic
  primer (1)..(32): yccV forward primer
attcatatguggttataaagacatcaacatgc

SEQ ID NO: 113 - DNA, 90 bp, synthetic
  primer (1)..(90): yccV reverse primer
  misc_feature (65)..(65): n is a, c, g, or t
atccccattacgtgaggatggctaaggtccagtgaagtaccctgggcaaagagtttcataccttncaagtagtcacctcccgggaaatct

SEQ ID NO: 114 - DNA, 32 bp, synthetic
  primer (1)..(32): ycjX forward primer
attcatatguttggctgatactgtaattcttc

SEQ ID NO: 115 - DNA, 90 bp, synthetic
  primer (1)..(90): ycjX reverse primer
  misc_feature (65)..(65): n is a, c, g, or t
atccccattacgtgaggatggctaaggtccagtgaagtaccctgggcaaagagtttcataccttncaagttgctgtcctgtgctgctctg

SEQ ID NO: 116 - DNA, 32 bp, synthetic
  primer (1)..(32): mutM forward primer
attcatatguggcgaaaagtactaagtactta

SEQ ID NO: 117 - DNA, 90 bp, synthetic
  primer (1)..(90): mutM reverse primer
  misc_feature (65)..(65): n is a, c, g, or t
atccccattacgtgaggatggctaaggtccagtgaagtaccctgggcaaagagtttcataccttncaagtagcatctccaggaatgaaca

SEQ ID NO: 118 - DNA, 19 bp, synthetic
  primer (1)..(19): primer P492
tgcaactcttcttcaacgc

SEQ ID NO: 119 - DNA, 19 bp, synthetic
  primer (1)..(19): primer P493
aagaaccaggcgcttctaa

SEQ ID NO: 120 - DNA, 19 bp, synthetic
  primer (1)..(19): primer P525
attgatgacctgatggcac

SEQ ID NO: 121 - DNA, 18 bp, synthetic
  primer (1)..(18): primer P526
gatccagacttcgaagcg

SEQ ID NO: 122 - DNA, 90 bp, synthetic
  primer (1)..(90): ibpA forward primer
  misc_feature (65)..(65): n is a, c, g, or t
atccccattacgtgaggatggctaaggtccagtgaagtaccctgggcaaagagtttcataccttncaagtaatcaatagctcctgaaatc

SEQ ID NO: 123 - DNA, 31 bp, synthetic
  primer (1)..(31): ibpA reverse primer
attcatatgtttggcctgatgagttatagcg

SEQ ID NO: 124 - DNA, 32 bp, synthetic
  primer (1)..(32): grpE forward primer
attcatatgutctccgcgagcgtgccagtttt

SEQ ID NO: 125 - DNA, 90 bp, synthetic
  primer (1)..(90): grpE reverse primer
  misc_feature (65)..(65): n is a, c, g, or t
atccccattacgtgaggatggctaaggtccagtgaagtaccctgggcaaagagtttcataccttncaagtgaatttctccgcgttttttt

SEQ ID NO: 126 - DNA, 32 bp, synthetic
  primer (1)..(32): ldhA forward primer
attcatatgugggaacccacagcccgagcgtc

SEQ ID NO: 127 - DNA, 90 bp, synthetic
  primer (1)..(90): ldhA reverse primer
  misc_feature (65)..(65): n is a, c, g, or t
atccccattacgtgaggatggctaaggtccagtgaagtaccctgggcaaagagtttcataccttncaagtaagactttctccagtgatgt

SEQ ID NO: 128 - DNA, 122 bp, synthetic
  primer (1)..(122): ybbN forward primer
  misc_feature (97)..(97): n is a, c, g, t or u
attcatatgucccattcgtactcgcttcaccgatccccattacgtgaggatggctaaggtccagtgaagtaccctgggcaaagagtttcataccttncaagtggagtcgctctctgttgtcg

SEQ ID NO: 129 - DNA, 90 bp, synthetic
  primer (1)..(90): ybbN reverse primer
  misc_feature (65)..(65): n is a, c, g, or t
atccccattacgtgaggatggctaaggtccagtgaagtaccctgggcaaagagtttcataccttncaagtggagtcgctctctgttgtcg

SEQ ID NO: 130 - DNA, 32 bp, synthetic
  primer (1)..(32): fxsA forward primer
attcatatgutaaacacacagaatatatgtgg

SEQ ID NO: 131 - DNA, 90 bp, synthetic
  primer (1)..(90): fxsA reverse primer
  misc_feature (65)..(65): n is a, c, g, or t
atccccattacgtgaggatggctaaggtccagtgaagtaccctgggcaaagagtttcataccttncaagtaggtttctcctgtaatagca

SEQ ID NO: 132 - DNA, 31 bp, synthetic
  primer (1)..(31): rrnB forward primer
attcatatgugcaaacacgccgccgggtcag

SEQ ID NO: 133 - DNA, 90 bp, synthetic
  primer (1)..(90): rrnB reverse primer
  misc_feature (65)..(65): n is a, c, g, or t
atccccattacgtgaggatggctaaggtccagtgaagtaccctgggcaaagagtttcataccttncaagtaaaagtttgacgctcaaaga

SEQ ID NO: 134 - DNA, 35 bp, synthetic
  primer (1)..(35): rrnE forward primer
attcatatguaatgcgcctccgttgagacgacaac

SEQ ID NO: 135 - DNA, 90 bp, synthetic
  primer (1)..(90): rrnE reverse primer
  misc_feature (65)..(65): n is a, c, g, or t
atccccattacgtgaggatggctaaggtccagtgaagtaccctgggcaaagagtttcataccttncaagtaaaagtttgatgctcaaaga

SEQ ID NO: 136 - DNA, 32 bp, synthetic
  primer (1)..(32): poxB forwrad primer
attcatatgutaggttgtcgctgcctgccgtg

SEQ ID NO: 137 - DNA, 90 bp, synthetic
  primer (1)..(90): poxB reverse primer
  misc_feature (65)..(65): n is a, c, g, or t
atccccattacgtgaggatggctaaggtccagtgaagtaccctgggcaaagagtttcataccttncaagtggttctccatctcctgaatg

SEQ ID NO: 138 - DNA, 32 bp, synthetic
  primer (1)..(32): cspD forward primer
attcatatgucggttatcggcagaacgccctg

SEQ ID NO: 139 - DNA, 90 bp, synthetic
  primer (1)..(90): cspD reverse primer
  misc_feature (65)..(65): n is a, c, g, or t
atccccattacgtgaggatggctaaggtccagtgaagtaccctgggcaaagagtttcataccttncaagtgcttcgacatccttcgcaaa

SEQ ID NO: 140 - DNA, 1902 bp, synthetic
  integration sequence s9_pmutM_folP (1)..(1902)
  CDS (299)..(1093): kanR
  promoter (1533)..(1832): burden sensing promoter p(mutM)
  RBS (1833)..(1838): rbs catalog
  misc_feature (1838)..(1838): n is a, c, g, or t
  gene (1844)..(1902): beginning of folP gene
aagaaccaggcgcttctaacaattctggcgacaatggtagtccaaaggctcctcgtccggttgatgaaccgcgtacgccgaacccgggtaacaccatgtcagagcagttaggcgacaagtaagttcccgcatcagatgactgtatttgtaccgaaaaccccggggcgtgctccggggttttttcttatcaattcataccagggataacatcagcgattgtgtaggctggagctgcttcgaagttcctatactttctagagaataggaacttcggaataggaacttcaagatccccttattagaagaactcgtcaagaaggcgatagaaggcgatgcgctgcgaatcgggagcggcgataccgtaaagcacgaggaagcggtcagcccattcgccgccaagctcttcagcaatatcacgggtagccaacgctatgtcctgatagcggtccgccacacccagccggccacagtcgatgaatccagaaaagcggccattttccaccatgatattcggcaagcaggcatcgccatgggtcacgacgagatcctcgccgtcgggcatgcgcgccttgagcctggcgaacagttcggctggcgcgagcccctgatgctcttcgtccagatcatcctgatcgacaagaccggcttccatccgagtacgtgctcgctcgatgcgatgtttcgcttggtggtcgaatgggcaggtagccggatcaagcgtatgcagccgccgcattgcatcagccatgatggatactttctcggcaggagcaaggtgagatgacaggagatcctgccccggcacttcgcccaatagcagccagtcccttcccgcttcagtgacaacgtcgagcacagctgcgcaaggaacgcccgtcgtggccagccacgatagccgcgctgcctcgtcctgcagttcattcagggcaccggacaggtcggtcttgacaaaaagaaccgggcgcccctgcgctgacagccggaacacggcggcatcagagcagccgattgtctgttgtgcccagtcatagccgaatagcctctccacccaagcggccggagaacctgcgtgcaatccatcttgttcaatcatgcgaaacgatcctcatcctgtctcttgatcagatcttgatcccctgcgccatcagatccttggcggcaagaaagccatccagtttactttgcagggcttcccaaccttaccagagggcgccccagctggcaattccggttcgcttgctgtccataaaaccgcccagtctagctatcgccatgtaagcccactgcaagctacctgctttctctttgcgcttgcgttttcccttgtccagatagcccagtagctgacattcatccggggtcagcaccgtttctgcggactggctttctacgtgttccgcttcctttagcagcccttgcgccctgagtgcttgcggcagcgtgagcttcaaaagcgctctgaagttcctatactttctagagaataggaacttcgaactgcaggtcgacggatccccggaatattcatatgtggcgaaaagtactaagtacttagaggaaataaatcatggctaaaggtattcgtgagaaaatcaagctggtttcttctgctggtactggtcacttctataccactacgaagaacaaacgtactaagccggaaaaactggaactgaaaaaattcgatccagttgttcgccagcacgtgatctacaaagaagcgaaaatcaaataattctcgctttgatgtaacaaaaaacctcgctccggcggggttttttgttatctgcttgcccccatattgactgcatctgttcattcctggagatgctacttgnaaggtatgaaactctttgcccagggtacttcactggaccttagccatcctcacgtaatggggat

SEQ ID NO: 141 - protein, 161 aa, synthetic
LEELVKKAIEGDALRIGSGDTVKHEEAVSPFAAKLFSNITGSQRYVLIAVRHTQPATVDESRKAAIFHHDIRQAGIAMGHDEILAVGHARLEPGEQFGWREPLMLFVQIILIDKTGFHPSTCSLDAMFRLVVEWAGSRIKRMQPPHCISHDGYFLGRSKVR

SEQ ID NO: 142 - protein, 10 aa, synthetic
QEILPRHFAQ

SEQ ID NO: 143 - protein, 25 aa, synthetic
QPVPSRFSDNVEHSCARNARRGQPR

SEQ ID NO: 144 - protein, 26 aa, synthetic
PRCLVLQFIQGTGQVGLDKKNRAPLR

SEQ ID NO: 145 - protein, 20 aa, synthetic
QPEHGGIRAADCLLCPVIAE

SEQ ID NO: 146 - protein, 18 aa, synthetic
PLHPSGRRTCVQSILFNH

SEQ ID NO: 147 - DNA, 1347 bp, Bacillus licheniformis
  CDS (1)..(1347): Bacillus licheniformis essential gene glmM
atgggcaagtattttggtacagacggtgtaagaggcgtggcaaacagtgaacttacacctgagctggcctttaaagtcggacgctttggcggatatgtcctaacaaaagataaggagcgtcccaaggttctgatcggccgtgacacgcgcatttcagggcatatgctggaaggggcccttgtagcaggccttctttcgataggagcagaagtcatgcgtctcggcgtgatttcgacgcccggagtcgcatatttgacgaaggctatggacgcggaggcgggtgtgatgatttccgcttcccacaaccctgtccaggacaacggaattaagtttttcggcggcgacggctttaagctttccgatgaacaggagcttgaaatcgagcgtctgatggatcagccggaagatcacctgccaaggcctgtaggcgctgatctgggcatggtgaacgactactttgaaggcggacagaaatatttgcagtttcttaagcagtctgctgatgaagacttcacaggcattcatgtcgcgcttgactgtgcgcacggggcgacatcttcgctggcgacccacctgtttgccgatcttgacgcagatgtatcgacgatggggacttctccgaacggattaaacatcaatgacggagtcggatcaacccaccctgaagccctggcagaatttgtgaaggaaaagggagctgacgtcggcatggcgtttgacggggatggcgaccgcttaatcgctgtcgacgaaaaagggaatatcgtagacggcgatcaaatcatgtacatatgcgcgaagtacttgaagagcgaggggcgcctgacggacaataccgttgtctccacggtgatgagcaacctcggtttctacaaagcgcttgaagcggaaggcattaaaagcgttcagacagcggtcggcgaccgctatgtagtggaggcgatgaaaaagggcggatttaccctcggcggagaacagtcgggacacctgattttccttgattacaatacgacaggcgacggactgctttctgcgatcatgctgatgaacacgattaaaatgacaggcaagccgctgtctgagcttgcggcagagatgcagaagtttccgcagctcctcttgaatgtgaaagtaaccgataaacataaagtaacggaaaacgaaaaggtaaaagcggtcatcgaagaagttgagaaggaaatgaacggtgacggccgcatccttgtgcgcccatccggcaccgagccgcttgtccgtgtcatggctgaagcgaaaacgaaggagctttgcgagaagtacgtaggccgcattgcagatgtcgtgaaagctgaaatgggagcagagtaa

SEQ ID NO: 148 - protein, 448 aa, Bacillus licheniformis
MGKYFGTDGVRGVANSELTPELAFKVGRFGGYVLTKDKERPKVLIGRDTRISGHMLEGALVAGLLSIGAEVMRLGVISTPGVAYLTKAMDAEAGVMISASHNPVQDNGIKFFGGDGFKLSDEQELEIERLMDQPEDHLPRPVGADLGMVNDYFEGGQKYLQFLKQSADEDFTGIHVALDCAHGATSSLATHLFADLDADVSTMGTSPNGLNINDGVGSTHPEALAEFVKEKGADVGMAFDGDGDRLIAVDEKGNIVDGDQIMYICAKYLKSEGRLTDNTVVSTVMSNLGFYKALEAEGIKSVQTAVGDRYVVEAMKKGGFTLGGEQSGHLIFLDYNTTGDGLLSAIMLMNTIKMTGKPLSELAAEMQKFPQLLLNVKVTDKHKVTENEKVKAVIEEVEKEMNGDGRILVRPSGTEPLVRVMAEAKTKELCEKYVGRIADVVKAEMGAE

SEQ ID NO: 149 - DNA, 282 bp, Bacillus licheniformis
  CDS (1)..(282): Bacillus licheniformis essential gene ylaN
ttggcgtctgagattgtagtcgaccatcgtgaaaaagcacttgctctgttaaaacgtgatgctgataaaatcttaaagctgattcaagtgcaaatggacaacttaacgatgcctcaatgtcctctttatgaagaggttttagatacacaaatgttcggactctctagagaaattgattttgctgtccgccttggattagtggatgaagaagagggtaaagaactgctttacaggctggagcgtgaattgtctgcattacatgatgcatttacaaaaaaataa

SEQ ID NO: 150 - protein, 93 aa, Bacillus licheniformis
LASEIVVDHREKALALLKRDADKILKLIQVQMDNLTMPQCPLYEEVLDTQMFGLSREIDFAVRLGLVDEEEGKELLYRLERELSALHDAFTKK

SEQ ID NO: 151 - DNA, 219 bp, Bacillus licheniformis
  CDS (1)..(219): Bacillus licheniformis essential gene infA
atggcgaaagacgatgtaattgaagtggaaggtactgtagtcgaaacgctgccaaacgcaatgttcaaagttgaacttgagaatggccacacggttttggctcacgtatctggtaaaatccgcatgcacttcattcgcattttacctggagacaaagttacggtagaattatctccatatgacttaactcgtggtagaattacgtaccgttacaaataa

SEQ ID NO: 152 - protein, 72 aa, Bacillus licheniformis
MAKDDVIEVEGTVVETLPNAMFKVELENGHTVLAHVSGKIRMHFIRILPGDKVTVELSPYDLTRGRITYRYK

SEQ ID NO: 153 - DNA, 870 bp, Bacillus licheniformis
  CDS (1)..(870): Bacillus licheniformis essential gene dapA
atgaacttcggaaatatcgcaaccgcgatggttacgccctttgacaaaaatgaaaatatcgattttcaaaaactgtcaaagctgatcgattatttactaaacaatgggacggattccctggtcgttgccggaacaaccggagaatcgccgacgctttccgaagaagaaaaggtagcgctcattcaatactctgtcaaggaagcggcaggccgtgccccaatcatcgccggcacgggaagcaacaacacgaaggcgtcgatcaagctgacgaaaaaagctgaagaagccggcgctgacgctgtcatgctcgtcactccgtactacaacaagccttctcaggaaggcatgtaccgccatttcagagcgattgcggaggaaacatcgctgcctgtcatgctttataatgtgccgggaagaacggctgcttcgctcgcaccagagacgacaatccgccttgcggagatcccgaatattatcgccattaaagaagcgagcggcgacctagatgcgataacaaaaatcgtagccgaaacccctgaggactttgcagtttattcaggagatgacagcctgacactgccggcgctgtccgtgggagcgagaggaatcgtttccgttgcatcacacatcatcggaccggaaatgcaggaaatgatcaaacattataccgaggggaacacggctcaggctgctttgatccatcaaaagctgcttccgctgatgaaagggctttttgccgcaccgaacccgtctccattaaagacggctcttcagctgaagggtcttgacgtcgggtccgtccggctccctttgattccgctaaatgaagatgaacgactccgtttaagcagcctgatgaacggcctgtaa

SEQ ID NO: 154 - protein, 289 aa, Bacillus licheniformis
MNFGNIATAMVTPFDKNENIDFQKLSKLIDYLLNNGTDSLVVAGTTGESPTLSEEEKVALIQYSVKEAAGRAPIIAGTGSNNTKASIKLTKKAEEAGADAVMLVTPYYNKPSQEGMYRHFRAIAEETSLPVMLYNVPGRTAASLAPETTIRLAEIPNIIAIKEASGDLDAITKIVAETPEDFAVYSGDDSLTLPALSVGARGIVSVASHIIGPEMQEMIKHYTEGNTAQAALIHQKLLPLMKGLFAAPNPSPLKTALQLKGLDVGSVRLPLIPLNEDERLRLSSLMNGL

SEQ ID NO: 155 - DNA, 2830 bp, synthetic
  promoter (1)..(1000): pAOX1 promoter
  misc_feature (1)..(2830): pAOX1-ALB construct
  CDS (1001)..(2830): cds encoding Human_serum_albumin (hAS) protein
atgttggtattgtgaaatagacgcagatcgggaacactgaaaaataacagttattattcgagatctaacatccaaagacgaaaggttgaatgaaacctttttgccatccgacatccacaggtccattctcacacataagtgccaaacgcaacaggaggggatacactagcagcagaccgttgcaaacgcaggacctccactcctcttctcctcaacacccacttttgccatcgaaaaaccagcccagttattgggcttgattggagctcgctcattccaattccttctattaggctactaacaccatgactttattagcctgtctatcctggcccccctggcgaggttcatgtttgtttatttccgaatgcaacaagctccgcattacacccgaacatcactccagatgagggctttctgagtgtggggtcaaatagtttcatgttccccaaatggcccaaaactgacagtttaaacgctgtcttggaacctaatatgacaaaagcgtgatctcatccaagatgaactaagtttggttcgttgaaatgctaacggccagttggtcaaaaagaaacttccaaaagtcggcataccgtttgtcttgtttggtattgattgacgaatgctcaaaaataatctcattaatgcttagcgcagtctctctatcgcttctgaaccccggtgcacctgtgccgaaacgcaaatggggaaacacccgctttttggatgattatgcattgtctccacattgtatgcttccaagattctggtgggaatactgctgatagcctaacgttcatgatcaaaatttaactgttctaacccctacttgacagcaatatataaacagaaggaagctgccctgtcttaaacctttttttttatcatcattattagcttactttcataattgcgactggttccaattgacaagcttttgattttaacgacttttaacgacaacttgagaagatcaaaaaacaactaattattcgaaacgatgaagtgggtaacctttatttcccttctttttctctttagctcggcttattccaggggtgtgtttcgtcgagatgcacacaagagtgaggttgctcatcggtttaaagatttgggagaagaaaatttcaaagccttggtgttgattgcctttgctcagtatcttcagcagtgtccatttgaagatcatgtaaaattagtgaatgaagtaactgaatttgcaaaaacatgtgttgctgatgagtcagctgaaaattgtgacaaatcacttcataccctttttggagacaaattatgcacagttgcaactcttcgtgaaacctatggtgaaatggctgactgctgtgcaaaacaagaacctgagagaaatgaatgcttcttgcaacacaaagatgacaacccaaacctcccccgattggtgagaccagaggttgatgtgatgtgcactgcttttcatgacaatgaagagacatttttgaaaaaatacttatatgaaattgccagaagacatccttacttttatgccccggaactccttttctttgctaaaaggtataaagctgcttttacagaatgttgccaagctgctgataaagctgcctgcctgttgccaaagctcgatgaacttcgggatgaagggaaggcttcgtctgccaaacagagactcaagtgtgccagtctccaaaaatttggagaaagagctttcaaagcatgggcagtagctcgcctgagccagagatttcccaaagctgagtttgcagaagtttccaagttagtgacagatcttaccaaagtccacacggaatgctgccatggagatctgcttgaatgtgctgatgacagggcggaccttgccaagtatatctgtgaaaatcaagattcgatctccagtaaactgaaggaatgctgtgaaaaacctctgttggaaaaatcccactgcattgccgaagtggaaaatgatgagatgcctgctgacttgccttcattagctgctgattttgttgaaagtaaggatgtttgcaaaaactatgctgaggcaaaggatgtcttcctgggcatgtttttgtatgaatatgcaagaaggcatcctgattactctgtcgtgctgctgctgagacttgccaagacatatgaaaccactctagagaagtgctgtgccgctgcagatcctcatgaatgctatgccaaagtgttcgatgaatttaaacctcttgtggaagagcctcagaatttaatcaaacaaaattgtgagctttttgagcagcttggagagtacaaattccagaatgcgctattagttcgttacaccaagaaagtaccccaagtgtcaactccaactcttgtagaggtctcaagaaacctaggaaaagtgggcagcaaatgttgtaaacatcctgaagcaaaaagaatgccctgtgcagaagactatctatccgtggtcctgaaccagttatgtgtgttgcatgagaaaacgccagtaagtgacagagtcaccaaatgctgcacagaatccttggtgaacaggcgaccatgcttttcagctctggaagtcgatgaaacatacgttcccaaagagtttaatgctgaaacattcaccttccatgcagatatatgcacactttctgagaaggagagacaaatcaagaaacaaactgcacttgttgagctcgtgaaacacaagcccaaggcaacaaaagagcaactgaaagctgttatggatgatttcgcagcttttgtagagaagtgctgcaaggctgacgataaggagacctgctttgccgaggagggtaaaaaacttgttgctgcaagtcaagctgccttaggcttataa

SEQ ID NO: 156 - protein, 609 aa, synthetic [sequence omitted]

SEQ ID NO: 157 - DNA, 3505 bp, synthetic
  misc_feature (1)..(3505): construct KU70(up)-pPDI1-kanMX-terminator-KU70
  misc_feature (1)..(1002): upstream region
  promoter (1002)..(1542): promoter pPDI1
  CDS (1543)..(2352): kanMX
  terminator (2353)..(2555): terminator
  misc_feature (2556)..(3505): downstream region
gctcttcagaagcctaactttaatggggtaaaatatcagcagtaggctgaatatagagcatggcaacgtttacgtcaacagagtttaatagtgaaaactacgataggttcaggcctgtatacccagacgagttgtatcagcaattagtggattatcatgttggtgctaaaggattgtgtgtcgatgttggatgtggctctggccaggcaacgttcaccctgaaaaagtactttgacaaggtcataggatctgatatctcagaaaatcagttggcagtggctaggaaaagacagcctgctggaattgaatttaggttaggaacgggcgaggatttttcttggctaacggagacgccagatgtaatcaccgccgctgaatgcctgcactgggtagacccacagaaattcgttgcaaatgtcgccaattctctaagggatcatggcaccttgagttactggctttatacagaaccaatttttcagaacgaaagggccaatcaggtttacaacaaattcacctacgggtctgactacctgggcccatattgggatcctggccgtacacatttcagaaatcatttaaaggagttgaatcacatcttactggatagcgagctttttgacgaagtgaaaatttctaattttaaacaagaggaaggggtcaaaaacggagatatcttatacttggaaaaagagatgacaatcagtgatttcatcaattttgtatctagttggccttctgtgttttcgtggaagcagcaacgaggaaaggagggtatcctagatgatttttacaacgaactgaacgactgctttgaggggggtaacatgaaagtaatatggaactccgtcctagtatttgccaggaggaagcaaagggttgtataggctttagtacttatagaggaaacggggttacgtgcaagcgcgcatgcctgagctttgaggggggggactttcacatctcttcttctcacacttagccctaacacagagatcaactactcaaggcagcaccaaaagacgccagaaattatatggtccaggaaaaaacaactctctttactacaaaatttgaacaggtgtcctgcctgcggaaactacaaacgatcacacaccctctgcatgcattgcgtaggacaaatcaggagacattggaacgactctgttcctcaacaggaggcatttcgtgaagagtttgttaatcctttggatgagaagattctttatccaggaaagaaagaactgcccgatgaacgaactttacgtaagaaggagtggctgaagagaagaccccgaacactccctgttgaatagaacacgaacactgtaaatagaataaaagaaaacttggatagtagaacttcaatgtagtgtttctattgtcttacgcggctctttagattgcaatccccagaatggaatcgtccatctttctcaacccactcaaagataatctaccagacatacctacgccctccatcccagcaccacgtcgcgatcacccctaaaacttcaataattgaacacgtactgatttccaatgggtaaggaaaagactcacgtttcgaggccgcgattaaattccaacatggatgctgatttatatgggtataaatgggctcgcgataatgtcgggcaatcaggtgcgacaatctatcgattgtatgggaagcccgatgcgccagagttgtttctgaaacatggcaaaggtagcgttgccaatgatgttacagatgagatggtcagactaaactggctgacggaatttatgcctcttccgaccatcaagcattttatccgtactcctgatgatgcatggttactcaccactgcgatccccggcaaaacagcattccaggtattagaagaatatcctgattcaggtgaaaatattgttgatgcgctggcagtgttcctgcgccggttgcattcgattcctgtttgtaattgtccttttaacagcgatcgcgtatttcgtctcgctcaggcgcaatcacgaatgaataacggtttggttgatgcgagtgattttgatgacgagcgtaatggctggcctgttgaacaagtctggaaagaaatgcataagcttttgccattctcaccggattcagtcgtcactcatggtgatttctcacttgataaccttatttttgacgaggggaaattaataggttgtattgatgttggacgagtcggaatcgcagaccgataccaggatcttgccatcctatggaactgcctcggtgagttttctccttcattacagaaacggctttttcaaaaatatggtattgataatcctgatatgaataaattgcagtttcatttgatgctcgatgagtttttctaatcagtactgacaataaaaagattcttgttttcaagaacttgtcatttgtatagtttttttatattgtagttgttctattttaatcaaatgttagcgtgatttatattttttttcgcctcgacatcatctgcccagatgcgaagttaagtgcgcagaaagtaatatcatgcgtcaatcgtatgtgaatgctggtcgctatactgttcatcttagagaatgtcagtgaggttatttctgagctaatcattaccttgcccggtacaggaatagggtgttaccttattaattacgacggtggtcaaaacgacgaaatttaccccatttttgagttacaagacctgaatttggaaatgatgaaacaattgtaccaagtcttggaggaccatgtaagtgggcttaatcctctcgagaagcaattcccaattgaacacagtaaaccgttatcagccactctgttctttcacttaaggtctcttttttacatggcgaagactcataagcgtactggaagacattacaacttgaaaaagattttcttgttcactaataacgataaaccttacaatggaaactctcagctgagagttcccttgaagaaaaccctggctgattacaatgacgtagacattactttgattccgtttcttctgaacaagccttcaggtgtcaagtttgacaagacggaatactcagaaattttgttctatgataaagatgcttgttcgatgtcaattgaggagatccgccaacgaatttctagacataaggagatcaagcgggtttacttcacctgtcctttgaaaatcgcaaataacttgtgcatttctgtgaaaggttattctatgttttatcatgaaactccaaggaagatcaaatttgtcgtcaatgagggttcaactttcaaagatgtggagacaaaatctcagtttgtcgatccaacatccggaaaagagttttccagtgaacagctgatcaaagcatatcctctaggtgccgatgcttacattcctttaaactcagagcaagtcaaaacaataaatcgatttaatgatatcatcaatatcccctctttggaaattctaggtttcagggatatatctaattggttgccacagtatcagtttggcaaagcatcgtttttatcccctaataa

SEQ ID NO: 158 - protein, 269 aa, synthetic
MGKEKTHVSRPRLNSNMDADLYGYKWARDNVGQSGATIYRLYGKPDAPELFLKHGKGSVANDVTDEMVRLNWLTEFMPLPTIKHFIRTPDDAWLLTTAIPGKTAFQVLEEYPDSGENIVDALAVFLRRLHSIPVCNCPFNSDRVFRLAQAQSRMNNGLVDASDFDDERNGWPVEQVWKEMHKLLPFSPDSVVTHGDFSLDNLIFDEGKLIGCIDVGRVGIADRYQDLAILWNCLGEFSPSLQKRLFQKYGIDNPDMNKLQFHLMLDEFF

SEQ ID NO: 159 - DNA, 3533 bp, synthetic
  misc_feature (1)..(3533): KU70(up)-pFPR2-kanMX-terminator-KU70 construct
  misc_feature (1)..(1002): KU70 upstream region
  promoter (1003)..(1570): promoter pFPR2
  CDS (1571)..(2380): kanMX
  terminator (2381)..(2583): terminator
  misc_feature (2584)..(3533): KU70 downstream region
gctcttcagaagcctaactttaatggggtaaaatatcagcagtaggctgaatatagagcatggcaacgtttacgtcaacagagtttaatagtgaaaactacgataggttcaggcctgtatacccagacgagttgtatcagcaattagtggattatcatgttggtgctaaaggattgtgtgtcgatgttggatgtggctctggccaggcaacgttcaccctgaaaaagtactttgacaaggtcataggatctgatatctcagaaaatcagttggcagtggctaggaaaagacagcctgctggaattgaatttaggttaggaacgggcgaggatttttcttggctaacggagacgccagatgtaatcaccgccgctgaatgcctgcactgggtagacccacagaaattcgttgcaaatgtcgccaattctctaagggatcatggcaccttgagttactggctttatacagaaccaatttttcagaacgaaagggccaatcaggtttacaacaaattcacctacgggtctgactacctgggcccatattgggatcctggccgtacacatttcagaaatcatttaaaggagttgaatcacatcttactggatagcgagctttttgacgaagtgaaaatttctaattttaaacaagaggaaggggtcaaaaacggagatatcttatacttggaaaaagagatgacaatcagtgatttcatcaattttgtatctagttggccttctgtgttttcgtggaagcagcaacgaggaaaggagggtatcctagatgatttttacaacgaactgaacgactgctttgaggggggtaacatgaaagtaatatggaactccgtcctagtatttgccaggaggaagcaaagggttgtataggctttagtacttatagaggaaacggggttacgtgcaagcgcgcatgcctgagctttgaggggggggactttcacatctcttcttctcacacttagccctaacacagagatcaactacaagcggcaattcctacagaaagtgtttgcaaagttcctaatctcggtttgtcaccaagtcacttttctacgaaccctgagtttcctcacgaggaatcaagttttgaaatgcccgatttgtcgcagtttgatagttttgatgaattttttaatggaatctttccagaatttaaaagagtcaagaatatttaacttgtgagcgaacgaacatgaaaaccgaaagaatagttgatgatgatgttgaagcaatgcaagtaccatataaattaggagaagtcctttgtgtattggcgattccttttgatgcaagtgagcgtaaatggttaacaggctgatacatttactcaagctagtagtgaaagccattgcgaaatcagtttatcatagtagtggacgtcacaatggaactcatctctgcgaatcgttgtagaataactgtaggtaaatatgcaattctaacttctggtctaaaatgttcagtgacaatgcttatttctgtagtcgcgaagaattgcttctgaggagacggagcgagccatgtattctcgccaacttgacaagaacgccatgggtaaggaaaagactcacgtttcgaggccgcgattaaattccaacatggatgctgatttatatgggtataaatgggctcgcgataatgtcgggcaatcaggtgcgacaatctatcgattgtatgggaagcccgatgcgccagagttgtttctgaaacatggcaaaggtagcgttgccaatgatgttacagatgagatggtcagactaaactggctgacggaatttatgcctcttccgaccatcaagcattttatccgtactcctgatgatgcatggttactcaccactgcgatccccggcaaaacagcattccaggtattagaagaatatcctgattcaggtgaaaatattgttgatgcgctggcagtgttcctgcgccggttgcattcgattcctgtttgtaattgtccttttaacagcgatcgcgtatttcgtctcgctcaggcgcaatcacgaatgaataacggtttggttgatgcgagtgattttgatgacgagcgtaatggctggcctgttgaacaagtctggaaagaaatgcataagcttttgccattctcaccggattcagtcgtcactcatggtgatttctcacttgataaccttatttttgacgaggggaaattaataggttgtattgatgttggacgagtcggaatcgcagaccgataccaggatcttgccatcctatggaactgcctcggtgagttttctccttcattacagaaacggctttttcaaaaatatggtattgataatcctgatatgaataaattgcagtttcatttgatgctcgatgagtttttctaatcagtactgacaataaaaagattcttgttttcaagaacttgtcatttgtatagtttttttatattgtagttgttctattttaatcaaatgttagcgtgatttatattttttttcgcctcgacatcatctgcccagatgcgaagttaagtgcgcagaaagtaatatcatgcgtcaatcgtatgtgaatgctggtcgctatactgttcatcttagagaatgtcagtgaggttatttctgagctaatcattaccttgcccggtacaggaatagggtgttaccttattaattacgacggtggtcaaaacgacgaaatttaccccatttttgagttacaagacctgaatttggaaatgatgaaacaattgtaccaagtcttggaggaccatgtaagtgggcttaatcctctcgagaagcaattcccaattgaacacagtaaaccgttatcagccactctgttctttcacttaaggtctcttttttacatggcgaagactcataagcgtactggaagacattacaacttgaaaaagattttcttgttcactaataacgataaaccttacaatggaaactctcagctgagagttcccttgaagaaaaccctggctgattacaatgacgtagacattactttgattccgtttcttctgaacaagccttcaggtgtcaagtttgacaagacggaatactcagaaattttgttctatgataaagatgcttgttcgatgtcaattgaggagatccgccaacgaatttctagacataaggagatcaagcgggtttacttcacctgtcctttgaaaatcgcaaataacttgtgcatttctgtgaaaggttattctatgttttatcatgaaactccaaggaagatcaaatttgtcgtcaatgagggttcaactttcaaagatgtggagacaaaatctcagtttgtcgatccaacatccggaaaagagttttccagtgaacagctgatcaaagcatatcctctaggtgccgatgcttacattcctttaaactcagagcaagtcaaaacaataaatcgatttaatgatatcatcaatatcccctctttggaaattctaggtttcagggatatatctaattggttgccacagtatcagtttggcaaagcatcgtttttatcccctaataa

SEQ ID NO: 160 - protein, 269 aa, synthetic; identical to SEQ ID NO: 158

SEQ ID NO: 161 - DNA, 3632 bp, synthetic
  misc_feature (1)..(3632): construct KU70(up)-pRPL3-kanMX-terminator-KU70(dw)
  misc_feature (1)..(1002): KU70 upstream region
  promoter (1003)..(1669): pRPL3 promoter
  CDS (1670)..(2479): kanMX
  terminator (2480)..(2682): terminator
  misc_feature (2480)..(2682): KU70 downstream region
gctcttcagaagcctaactttaatggggtaaaatatcagcagtaggctgaatatagagcatggcaacgtttacgtcaacagagtttaatagtgaaaactacgataggttcaggcctgtatacccagacgagttgtatcagcaattagtggattatcatgttggtgctaaaggattgtgtgtcgatgttggatgtggctctggccaggcaacgttcaccctgaaaaagtactttgacaaggtcataggatctgatatctcagaaaatcagttggcagtggctaggaaaagacagcctgctggaattgaatttaggttaggaacgggcgaggatttttcttggctaacggagacgccagatgtaatcaccgccgctgaatgcctgcactgggtagacccacagaaattcgttgcaaatgtcgccaattctctaagggatcatggcaccttgagttactggctttatacagaaccaatttttcagaacgaaagggccaatcaggtttacaacaaattcacctacgggtctgactacctgggcccatattgggatcctggccgtacacatttcagaaatcatttaaaggagttgaatcacatcttactggatagcgagctttttgacgaagtgaaaatttctaattttaaacaagaggaaggggtcaaaaacggagatatcttatacttggaaaaagagatgacaatcagtgatttcatcaattttgtatctagttggccttctgtgttttcgtggaagcagcaacgaggaaaggagggtatcctagatgatttttacaacgaactgaacgactgctttgaggggggtaacatgaaagtaatatggaactccgtcctagtatttgccaggaggaagcaaagggttgtataggctttagtacttatagaggaaacggggttacgtgcaagcgcgcatgcctgagctttgaggggggggactttcacatctcttcttctcacacttagccctaacacagagatcaactccaacgacttgaggaaatgacgattatttcttaagatattcatggtgaggttttccaaatgtgatctgaaatgtaatcttggcaagtttggttcataaaacgtcaaaagaccacctgaagataaaaaataaagtggaaggagaagaaaaagaggtttttttccagatgagtctatgactaagatttctcttcaaagaattttttcaaggtttgagagggatgaaagcgaggctgctgcacgattatcgatgtcattcaatagggaggtagaagagaactgagggagaaaaggctacaactgaacctaaaactaactgaatttggaatgaagcctattacacgagaggtgtggcgcctttccaaagtcatcaggttcaagttattgctttctggagcaataaatgatgtcaatcccatacggggtctccacccttatagaattacttatctaccggctaggtgttgcatcgcggaccagcccaatcgggtaattttagttgaaaaggtttttagcgcgagtctagttattacccggatagtctaatgctgaaaatttctcggacatttttgatccgtacgtatatttcagtacggagaatcatcaacaagaatctttcaatgccaccaaaaaaaaagacatttttcaccatcgcgcattcacagtagcatgggtaaggaaaagactcacgtttcgaggccgcgattaaattccaacatggatgctgatttatatgggtataaatgggctcgcgataatgtcgggcaatcaggtgcgacaatctatcgattgtatgggaagcccgatgcgccagagttgtttctgaaacatggcaaaggtagcgttgccaatgatgttacagatgagatggtcagactaaactggctgacggaatttatgcctcttccgaccatcaagcattttatccgtactcctgatgatgcatggttactcaccactgcgatccccggcaaaacagcattccaggtattagaagaatatcctgattcaggtgaaaatattgttgatgcgctggcagtgttcctgcgccggttgcattcgattcctgtttgtaattgtccttttaacagcgatcgcgtatttcgtctcgctcaggcgcaatcacgaatgaataacggtttggttgatgcgagtgattttgatgacgagcgtaatggctggcctgttgaacaagtctggaaagaaatgcataagcttttgccattctcaccggattcagtcgtcactcatggtgatttctcacttgataaccttatttttgacgaggggaaattaataggttgtattgatgttggacgagtcggaatcgcagaccgataccaggatcttgccatcctatggaactgcctcggtgagttttctccttcattacagaaacggctttttcaaaaatatggtattgataatcctgatatgaataaattgcagtttcatttgatgctcgatgagtttttctaatcagtactgacaataaaaagattcttgttttcaagaacttgtcatttgtatagtttttttatattgtagttgttctattttaatcaaatgttagcgtgatttatattttttttcgcctcgacatcatctgcccagatgcgaagttaagtgcgcagaaagtaatatcatgcgtcaatcgtatgtgaatgctggtcgctatactgttcatcttagagaatgtcagtgaggttatttctgagctaatcattaccttgcccggtacaggaatagggtgttaccttattaattacgacggtggtcaaaacgacgaaatttaccccatttttgagttacaagacctgaatttggaaatgatgaaacaattgtaccaagtcttggaggaccatgtaagtgggcttaatcctctcgagaagcaattcccaattgaacacagtaaaccgttatcagccactctgttctttcacttaaggtctcttttttacatggcgaagactcataagcgtactggaagacattacaacttgaaaaagattttcttgttcactaataacgataaaccttacaatggaaactctcagctgagagttcccttgaagaaaaccctggctgattacaatgacgtagacattactttgattccgtttcttctgaacaagccttcaggtgtcaagtttgacaagacggaatactcagaaattttgttctatgataaagatgcttgttcgatgtcaattgaggagatccgccaacgaatttctagacataaggagatcaagcgggtttacttcacctgtcctttgaaaatcgcaaataacttgtgcatttctgtgaaaggttattctatgttttatcatgaaactccaaggaagatcaaatttgtcgtcaatgagggttcaactttcaaagatgtggagacaaaatctcagtttgtcgatccaacatccggaaaagagttttccagtgaacagctgatcaaagcatatcctctaggtgccgatgcttacattcctttaaactcagagcaagtcaaaacaataaatcgatttaatgatatcatcaatatcccctctttggaaattctaggtttcagggatatatctaattggttgccacagtatcagtttggcaaagcatcgtttttatcccctaataa

SEQ ID NO: 162 - protein, 269 aa, synthetic; identical to SEQ ID NO: 158

SEQ ID NO: 163 - DNA, 3573 bp, synthetic
  misc_feature (1)..(3573): construct KU70(up)-pRPL6A-kanMX-terminator-KU70(dw)
  misc_feature (1)..(1002): KU70 upstream region
  promoter (1003)..(1610): promoter pRPL6A
  CDS (1611)..(2420): kanMX
  terminator (2421)..(2623): terminator
  misc_feature (2624)..(3573): KU70 downstream region
gctcttcagaagcctaactttaatggggtaaaatatcagcagtaggctgaatatagagcatggcaacgtttacgtcaacagagtttaatagtgaaaactacgataggttcaggcctgtatacccagacgagttgtatcagcaattagtggattatcatgttggtgctaaaggattgtgtgtcgatgttggatgtggctctggccaggcaacgttcaccctgaaaaagtactttgacaaggtcataggatctgatatctcagaaaatcagttggcagtggctaggaaaagacagcctgctggaattgaatttaggttaggaacgggcgaggatttttcttggctaacggagacgccagatgtaatcaccgccgctgaatgcctgcactgggtagacccacagaaattcgttgcaaatgtcgccaattctctaagggatcatggcaccttgagttactggctttatacagaaccaatttttcagaacgaaagggccaatcaggtttacaacaaattcacctacgggtctgactacctgggcccatattgggatcctggccgtacacatttcagaaatcatttaaaggagttgaatcacatcttactggatagcgagctttttgacgaagtgaaaatttctaattttaaacaagaggaaggggtcaaaaacggagatatcttatacttggaaaaagagatgacaatcagtgatttcatcaattttgtatctagttggccttctgtgttttcgtggaagcagcaacgaggaaaggagggtatcctagatgatttttacaacgaactgaacgactgctttgaggggggtaacatgaaagtaatatggaactccgtcctagtatttgccaggaggaagcaaagggttgtataggctttagtacttatagaggaaacggggttacgtgcaagcgcgcatgcctgagctttgaggggggggactttcacatctcttcttctcacacttagccctaacacagagatcaactcgcttcagcatttcgacagtgtaaagaagctcatctcacttgaccagaatgcttttgctatctgttatttcaaagacctagagtacctcccaattgccatagaagcttggaaactttatgaaccttcttctaaagtaccggtggtattcgctcaagtgacacaactccccaaatcagctccaatcgaatggagcgggtcagtgtatcaagagacaccaaactacgatgattactacggtgattcgtcagaaaatgaagatgagtccacacagattgccaacaacttgtcctcgctagaattacagggacaatcggtcacatttcaagacggctacgttagcttgacattcgccccaggcctatcagccacagcacacaacacggtaattttaaacaaggggcaggcaagcaagctggaaaccattccacaggaatattccgtcgacatcatccccgtcaacagactgttcgatttcacagggaaagatcaggacctagccgtactccacaggctgaacatctgagatcaggcatgagaatccttacaccatctatgttgctctagggctgtcaaccctattatgcacgtgacggtgcgactctttcaaatgggtaaggaaaagactcacgtttcgaggccgcgattaaattccaacatggatgctgatttatatgggtataaatgggctcgcgataatgtcgggcaatcaggtgcgacaatctatcgattgtatgggaagcccgatgcgccagagttgtttctgaaacatggcaaaggtagcgttgccaatgatgttacagatgagatggtcagactaaactggctgacggaatttatgcctcttccgaccatcaagcattttatccgtactcctgatgatgcatggttactcaccactgcgatccccggcaaaacagcattccaggtattagaagaatatcctgattcaggtgaaaatattgttgatgcgctggcagtgttcctgcgccggttgcattcgattcctgtttgtaattgtccttttaacagcgatcgcgtatttcgtctcgctcaggcgcaatcacgaatgaataacggtttggttgatgcgagtgattttgatgacgagcgtaatggctggcctgttgaacaagtctggaaagaaatgcataagcttttgccattctcaccggattcagtcgtcactcatggtgatttctcacttgataaccttatttttgacgaggggaaattaataggttgtattgatgttggacgagtcggaatcgcagaccgataccaggatcttgccatcctatggaactgcctcggtgagttttctccttcattacagaaacggctttttcaaaaatatggtattgataatcctgatatgaataaattgcagtttcatttgatgctcgatgagtttttctaatcagtactgacaataaaaagattcttgttttcaagaacttgtcatttgtatagtttttttatattgtagttgttctattttaatcaaatgttagcgtgatttatattttttttcgcctcgacatcatctgcccagatgcgaagttaagtgcgcagaaagtaatatcatgcgtcaatcgtatgtgaatgctggtcgctatactgttcatcttagagaatgtcagtgaggttatttctgagctaatcattaccttgcccggtacaggaatagggtgttaccttattaattacgacggtggtcaaaacgacgaaatttaccccatttttgagttacaagacctgaatttggaaatgatgaaacaattgtaccaagtcttggaggaccatgtaagtgggcttaatcctctcgagaagcaattcccaattgaacacagtaaaccgttatcagccactctgttctttcacttaaggtctcttttttacatggcgaagactcataagcgtactggaagacattacaacttgaaaaagattttcttgttcactaataacgataaaccttacaatggaaactctcagctgagagttcccttgaagaaaaccctggctgattacaatgacgtagacattactttgattccgtttcttctgaacaagccttcaggtgtcaagtttgacaagacggaatactcagaaattttgttctatgataaagatgcttgttcgatgtcaattgaggagatccgccaacgaatttctagacataaggagatcaagcgggtttacttcacctgtcctttgaaaatcgcaaataacttgtgcatttctgtgaaaggttattctatgttttatcatgaaactccaaggaagatcaaatttgtcgtcaatgagggttcaactttcaaagatgtggagacaaaatctcagtttgtcgatccaacatccggaaaagagttttccagtgaacagctgatcaaagcatatcctctaggtgccgatgcttacattcctttaaactcagagcaagtcaaaacaataaatcgatttaatgatatcatcaatatcccctctttggaaattctaggtttcagggatatatctaattggttgccacagtatcagtttggcaaagcatcgtttttatcccctaataa

SEQ ID NO: 164 - protein, 269 aa, synthetic; identical to SEQ ID NO: 158